European Patent Application EP 4 438 717 A1, published October 2, 2024. Title: ACID-RESISTANT YEAST STRAIN FOR HIGH-YIELD PRODUCTION OF SUCCINIC ACID, AND CONSTRUCTION METHOD THEREFOR AND USE THEREOF. Applicant: Tianjin Institute of Industrial Biotechnology, Chinese Academy of Sciences. The sequence listing filed with the application follows.

SEQUENCE LISTING (162 sequences)

SEQ ID NO: 1 - DNA, 1339 bp, synthetic construct
  misc_feature 1..1339: note = encoding Sorghum bicolor SbMDH
  source 1..1339: mol_type = other DNA
actaccacccccaacacaaacacaatgggtttgtctaccgcatactctccagttggttctcacttggctccagcaccattaggtcacagaagatccgctcaattacatagaccaagaagagcattgttagctaccgttagatgttccgttgatgctgcaaagcaagttcaagatggtgttgctactgcagaagctccagcaactagaaaggattctttcggtgttttctctactacctacgacttaaaggcagaagataagaccaagtcctggaagaagttggttaacattgctgtttctggtgcagctggtatgatttccaaccacttgttattcaagttggcttctggtgaagttttcggtcaagaccaaccaattgcattaaagttattgggttccgaaagatctttccaagctttggaaggtgttgctatggaattggaagattccttgtacccattattgagagaagtttccattggtattgacccatacgaagttttcgaagacgttgattgggcattattgattggtgctaagccaagaggtccaggtatggaaagagcagctttgttagacattaacggtcaaattttcgctgatcaaggtaaggcattgaacgctgttgcatctaagaacgttaaggttttggttgttggtaacccatgtaacaccaacgctttgatttgtttgaagaacgcaccagatattccagctaagaacttccacgcattaaccagattggacgaaaacagagcaaagtgtcaattggctttaaaggcaggtgttttctacgataaggtttccaacgttaccatttggggtaaccactctactacccaagttccagatttcttgaacgcaaagattgacggtagaccagttaaggaagttattaaggacactaagtggttggaagaagaattcaccattactgttcaaaagagaggtggtgctttgattcaaaagtggggtagatcctctgcagcttccaccgctgtttctattgctgacgcaattaagtccttggttaccccaactccagaaggtgactggttttccaccggtgtttacaccactggtaacccatacggtattgcagaagacattgttttctccatgccatgtagatctaagggtgatggtgactacgaattggcaaccgatgtttccatggacgatttcttatgggaaagaattaagaagtccgaagcagaattgttggcagaaaagaaggctgttgctcacttgaccggtgaaggtaacgcatactgtgacgttccagaagatactatgttgccaggtgaagtttaactacaacaagatgtttgttcaaggg

SEQ ID NO: 2 - DNA, 1373 bp, synthetic construct
  misc_feature 1..1373: note = encoding Schizosaccharomyces pombe SpMAE1
  source 1..1373: mol_type = other DNA
caaaacacacaaacaaacacaattacaaaaaatgggtgaattaaaggaaatcttaaagcaaagataccacgaattattggactggaatgtcaaggcaccacacgtcccattgtctcaaagattaaagcactttacttggtcttggttcgcttgtactatggcaaccggtggtgttggtttgattattggttccttcccattcagattctacggtttaaacaccatcggtaaaatcgtttacatcttgcaaattttcttgttctctttgtttggttcctgtatgttgttcagattcattaagtacccatctactattaaggattcctggaaccaccacttggaaaagttgtttattgcaacttgtttgttgtctatttccaccttcattgatatgttggctatctacgcatacccagacactggtgaatggatggtttgggttattagaatcttgtactacatctacgttgctgtttctttcatctactgtgttatggctttctttaccattttcaacaaccacgtttacactattgaaaccgcttctccagcatggattttaccaattttcccaccaatgatttgtggtgttattgctggtgcagttaactccactcaaccagctcatcaattgaagaacatggttattttcggtatcttgttccaaggtttgggtttttgggtttacttgttattgttcgcagttaacgttttaagattctttaccgttggtttggctaagccacaagacagaccaggtatgtttatgttcgttggtccaccagctttttctggtttagcattgattaacattgctagaggtgcaatgggttccagaccatacattttcgttggtgcaaactcttccgaatacttaggtttcgtttctacttttatggctattttcatttggggtttggctgcatggtgttactgtttagcaatggtttcctttttggctggtttctttactagagctccattgaagttcgcatgtggttggtttgctttcattttcccaaacgttggtttcgttaactgtaccatcgaaatcggtaaaatgatcgattctaaggcattccaaatgttcggtcacatcatcggtgttattttgtgtatccaatggatcttgttgatgtacttgatggttagagcatttttagttaacgacttgtgttaccctggtaaagatgaagacgctcacccaccaccaaagccaaacactggtgttttaaacccaaccttcccaccagaaaaggctccagcatccttggaaaaggttgatacccacgttacctctactggtggtgaatctgacccaccatcctctgaacacgaatccgtctaaatcactttctgtcaattgtcttaat

SEQ ID NO: 3 - DNA, 1466 bp, synthetic construct
  misc_feature 1..1466: note = encoding ScFRD
  source 1..1466: mol_type = other DNA
accccccctccccctattagaaaaaatgtccttgtctccagttgttgttattggtactggtttggcaggtttagctgcagctaacgaattggttaacaagtacaacattccagttaccattttagaaaaggcttcttccattggtggtaactctattaaggcatcttccggtattaacggtgcttgtactgaaacccaaagacacttccatattgaagactccccaagattgtttgaagatgacactattaagtctgcaaagggtaaaggtgttcaagaattgatggcaaagttagctaacgattccccattggctatcgaatggttgaagaacgaattcgatttgaagttagacttgttagcacaattaggtggtcactctgttgctagaactcatagatcttccggtaaattgccaccaggtttcgaaatcgtttccgcattgtctaacaacttgaagaagttagctgaaaccaagccagaattagttaagatcaacttggattccaaggttgttgacattcacgaaaaggatggttccatttctgcagttgtttacgaagacaagaacggtgaaaagcatatggtttctgctaacgatgttgttttctgttccggtggtttcggtttttctaaggaaatgttgaaggaatacgcaccagaattggttaacttaccaactaccaacggtcaacaaactaccggtgacggtcaaagattgttacaaaagttgggtgctgatttgatcgatatggaccaaatccaagttcacccaaccggtttcattgatccaaacgacagatcttcctcttggaagtttttggcagctgaatccttgagaggtttaggtggtattttgttaaacccaatcactggtagaagattcgttaacgaattaactaccagagacgttgttaccgcagctattcaaaaggtttgtccacaagaagataacagagcattgttagttatgggtgaaaagatgtacactgacttgaagaacaacttggatttctacatgtttaagaagttggttcaaaagttgaccttatcccaagttgtttctgaatacaacttgccaatcactgttgcacaattgtgtgaagaattacaaacctactcctctttcactaccaaggctgacccattgggtagaactgttatcttgaacgaattcggttctgatgttactccagaaaccgttgttttcattggtgaagttactccagttgttcactttaccatgggtggtgcaagaattaacgttaaggctcaagttattggtaaaaacgacgaaagattgttaaagggtttgtacgcagctggtgaagtttccggtggtgttcatggtgcaaacagattaggtggttcctctttgttagaatgtgttgttttcggtagaaccgcagctgaatctattgctaacgatagaaagtaagtctagagagtgtatacctccccgcttt

SEQ ID NO: 4 - DNA, 3488 bp, synthetic construct
  misc_feature 1..3488: note = encoding LmFRD
  source 1..3488: mol_type = other DNA
accccccctccccctattagaaaaaatggctgatggtaaaacttctgcatccgttgttgcagttgatgctgaaagagctgcaaaggaaagagacgctgcagctagagcaatgttgcaaggtggtggtgtttctccagctggtaaagctcaattgttaaagaagggtttggttcacactgttccatacaccttaaaggttgttgttgctgatccaaaggaaatggaaaaggcaactgctgacgcagaagaagttttacaagcagctttccaagttgttgataccttgttgaacaacttcaacgaaaactctgaagtttccagagttaacagattggctgttggtgaagaacaccaaatgtccgaaaccttaaagcatgttatggcatgttgtcaaaaggtttaccactcttccagaggtgtttttgacccagctgttggtccattagttagagaattgagagaagcagctcataagggtaaaactgttccagctgaaagagttaacgatttgttgtctaagtgtaccttgaacgcatctttctccattgacatgtccagaggtatgattgctagaaagcacccagatgcaatgttggacttaggtggtgttaacaagggttacggtatcgattacatcgttgaacatttgaactctttaggttacgatgacgttttctttgaatggggtggtgacgttagagcttctggtaaaaaccaattgtcccaaccatgggcagttggtattgttagaccaccagctttagcagatattagaactgttgttccagaagacaagagatcttttattagagttgttagattgaacaacgaagctattgcaacctccggtgactacgaaaacttagttgaaggtccaggttctaaggtttactcttccactttcaacccaacctccaagaacttgttagaaccaactgaagctggtatggctcaagtttctgttaagtgttgttcctgtatctacgctgacgcattggctaccgcagctttgttaaagaacgatccagcagctgttagaagaattttagacaactggagatacgttagagatactgttaccgactacactacctacactagagaaggtgaaagagttgctaagatgttggaaattgcaaccgaagatgctgaaatgagagcaaagagaattaagggttctttgccagctagagttattattgttggtggtggtttggcaggttgttccgcagctattgaagcagctaactgtggtgcacacgttatcttgttggaaaaggaaccaaagttaggtggtaactctgcaaaggctacttccggtattaacgcttggggtaccagagcacaagctaagcaaggtgttatggatggtggtaaattctttgaaagagacactcatagatctggtaaaggtggtaactgtgatccatgtttagttaagaccttgtctgttaagtcttccgacgctgttaagtggttgtccgaattaggtgttccattgactgttttatctcaattgggtggtgcttccagaaagagatgtcatagagcacctgataagtctgacggtaccccagttccagttggttttactattatgaagaccttggaaaaccacattgttaacgatttgtccagacatgttactgttatgaccggtattactgttaccgctttggaatctacttccagagttagaccagacggtgttttggttaagcacgttaccggtgttcacttgattcaagcttctggtcaatccatggttttgaacgcagatgctgttattttagcaactggtggtttttctaacgaccacaccccaaactccttgttacaacaatacgctccacaattgtcttccttcccaactaccaacggtgtttgggcaactggtgacggtgttaagatggcttctaagttaggtgttgcattggttgatatggacaaggttcaattacatccaactggtttgttagatccaaaggacccatctaacagaaccaagtacttaggtccagaagcattgagaggttccggtggtgttttgttaaacaagaacggtgaaagattcgttaacgaattggatttgagatctgttgtttcccaagcaattattgctcaagacaacgaatacccaggttctggtggttccaagtttgcttactgtgttttgaacgaaactgctgctaagttgttcggtaaaaacttcttgggtttctactggaacagattgggtttatttcaaaaggttgattctgttgcaggtttagcaaagttgattggttgtccagaagctaacgttgttgcaaccttaaagcaatacgaagaattatcttccaagaagttgaacccatgtccattaactggtaaatctgttttcccatgtgttttgggtacccaaggtccatactacgttgcattagttactccatccattcactacaccatgggtggttgtttgatttctccatccgctgaaatgcaaactattgataactctggtgttaccccagttagaagaccaattttgggtttatttggtgcaggtgaagttactggtggtgttcatggtggtaacagattgggtggtaactccttgttggaatgtgttgttttcggtaaaatcgctggtgacagagcagctactattttgcaaaagaagaacaccggtttatctatgactgaatggtccaccgttgttttaagagaagttagagaaggtggtgtttacggtgctggttctagagttttgagattcaacatgccaggtgctttacaaagaactggtttggcattaggtcaattcattggtattagaggtgactgggacggtcacagattgattggttactactctccaattaccttaccagatgacgttggtgttattggtattttggcaagagctgataagggtagattggctgaatggatttccgcattacaaccaggtgacgctgttgaaatgaaggcatgtggtggtttaatcatcgacagaagattcgctgaaagacacttctttttcagaggtcataagattagaaagttggctttaattggtggtggtaccggtgttgcaccaatgttgcaaattgttagagcagctgttaagaagccattcgttgattctatcgaatccatccaattcatctacgcagctgaagacgtttctgaattgacttacagaaccttgttagaatcttacgaagaagaatacggttccgaaaagtttaagtgtcatttcgttttgaacaacccaccagctcaatggactgatggtgttggtttcgttgacaccgcattgttaagatctgcagttcaagctccatccaacgatttgttagttgctatttgtggtccaccaattatgcaaagagctgttaagggtgcattaaagggtttgggttacaacatgaacttggttagaactgttgacgaaaccgaaccaccatcctaagtctagagagtgtatacctccccgcttt

SEQ ID NO: 5 - DNA, 3473 bp, synthetic construct
  misc_feature 1..3473: note = encoding TbFRD
  source 1..3473: mol_type = other DNA
accccccctccccctattagaaaaaatggttgatggtagatcttccgcatccattgttgctgttgatccagaaagagctgcaagagaaagagacgctgcagctagagctttgttacaagattccccattacacactaccatgcaatacgctacttctggtttggaattaaccgttccatacgcattgaaggttgttgcttctgcagatactttcgacagagcaaaggaagttgctgacgaagttttaagatgtgcatggcaattagctgataccgttttgaactcctttaacccaaactctgaagtttccttagttggtagattgccagttggtcaaaagcatcaaatgtctgctccattgaagagagttatggcatgttgtcaaagagtttacaactcttccgctggttgtttcgacccatccactgcaccagttgctaaggcattaagagaaattgcattgggtaaagaaagaaacaacgcatgtttggaagctttaactcaagcatgtaccttgccaaactctttcgttattgactttgaagctggtaccatttctagaaagcacgaacatgcatccttggatttgggtggtgtttctaagggttacatcgttgattacgttatcgacaacattaacgcagctggttttcaaaacgttttctttgattggggtggtgactgtagagcttccggtatgaacgcaagaaacactccatgggttgttggtattaccagaccaccatctttggatatgttaccaaacccaccaaaggaagcttcttacatctccgttatttctttggacaacgaagctttggcaacttctggtgactatgaaaacttaatctacaccgcagatgacaagccattgacttgtacctacgactggaagggtaaagaattaatgaagccatctcaatccaacattgctcaagtttctgttaagtgttactccgcaatgtacgctgatgcattggctactgcatgtttcattaagagagatccagctaaggttagacaattattagatggttggagatacgttagagataccgttagagactacagagtttacgttagagaaaacgaaagagttgcaaagatgtttgaaattgctactgaagatgcagaaatgagaaagagaagaatttccaacaccttgccagctagagttattgttgttggtggtggtttggcaggtttatctgcagctattgaagcagctggttgtggtgctcaagttgttttaatggaaaaggaagcaaagttgggtggtaactctgctaaggcaacttccggtattaacggttggggtaccagagctcaagcaaaggcttccattgttgatggtggtaaatacttcgaaagagacacttacaagtctggtattggtggtaacactgacccagctttagttaagaccttgtccatgaagtctgcagatgctattggttggttgacttctttaggtgttccattgaccgttttatctcaattgggtggtcactccagaaagagaactcatagagcaccagataagaaggacggtaccccattgccaattggtttcactattatgaagaccttagaagatcacgttagaggtaacttgtccggtagaattactattatggaaaactgttccgttacttctttgttatccgaaaccaaggaaagaccagacggtaccaagcaaattagagttactggtgttgaattcactcaagctggttctggtaaaactaccattttagcagatgctgttattttggcaactggtggtttctccaacgataagaccgctgactctttgttaagagaacacgcaccacatttggttaactttccaactaccaacggtccatgggctaccggtgacggtgttaagttagctcaaagattgggtgcacaattagttgatatggacaaggttcaattacatccaactggtttgattaacccaaaggatccagctaacccaaccaagttcttaggtccagaagcattgagaggttctggtggtgttttgttgaacaagcaaggtaaaagattcgttaacgaattggatttgagatctgttgtttccaaggctattatggaacaaggtgcagaatacccaggttctggtggttccatgttcgcttactgtgttttaaacgcagctgcacaaaagttgttcggtgtttcttcccacgaattttactggaagaagatgggtttatttgttaaggcagatactatgagagacttagctgcattgattggttgtccagttgaatccgttcaacaaaccttagaagaatacgaaagattgtctatttcccaaagatcctgtccaattactagaaagtctgtttacccatgtgttttgggtaccaagggtccatactacgttgctttcgttactccatctattcattacaccatgggtggttgtttaatttctccatccgctgaaattcaaatgaagaacacttcttccagagcaccattgtctcactccaacccaattttgggtttatttggtgctggtgaagttaccggtggtgttcatggtggtaacagattaggtggtaactctttgttagaatgtgttgttttcggtagaattgctggtgacagagcatccactattttacaaagaaagtcttccgcattgtcttttaaggtttggactaccgttgttttaagagaagttagagaaggtggtgtttacggtgctggttccagagttttgagattcaacttaccaggtgcattgcaaagatctggtttgtccttaggtcaattcattgctattagaggtgactgggacggtcaacaattgatcggttactactctccaatcactttaccagatgacttgggtatgattgatattttggctagatccgacaagggtaccttaagagaatggatttctgcattggaaccaggtgacgctgttgaaatgaaggcatgtggtggtttagttattgaaagaagattgtctgataagcacttcgtttttatgggtcatattattaacaagttgtgtttaattgctggtggtactggtgttgcaccaatgttgcaaattattaaggctgcattcatgaagccattcattgacaccttagaatccgttcacttgatctacgctgcagaagatgttactgaattaacctacagagaagttttggaagaaagaagaagagaatctagaggtaaattcaagaagactttcgttttgaacagaccaccaccattgtggaccgatggtgttggttttattgacagaggtattttaaccaaccatgttcaaccaccatctgacaacttgttagttgctatttgtggtccaccagttatgcaaagaatcgttaaggcaactttgaagaccttgggttacaacatgaacttggttagaactgttgatgaaaccgaaccatctggttcctaagtctagagagtgtatacctccccgcttt

SEQ ID NO: 6 - DNA, 3638 bp, synthetic construct
  misc_feature 1..3638: note = encoding AoPYC
  source 1..3638: mol_type = other DNA
caaaacacacaaacaaacacaattacaaaaaatggctgcaccattcagacaaccagaagaagctgttgatgacactgaattcattgatgaccaccatgaacacttgagagataccgttcaccatagattgagagcaaactcttccattatgcacttccaaaagattttagttgctaacagaggtgaaatcccaatcagaatttttagaactgcacatgaattgtccttacaaaccgttgctatctactcccatgaagacagattgtctatgcacagacaaaaggcagatgaagcttacatgattggtcacagaggtcaatacactccagttggtgcatacttagctggtgacgaaattattaagatcgcattggaacatggtgttcaattgattcacccaggttacggtttcttgtctgaaaacgcagattttgctagaaaggttgaaaacgctggtattgttttcgttggtccaactccagataccattgactccttaggtgacaaggtttctgcaagaagattggctattaagtgtgaagttccagttgttccaggtaccgaaggtccagttgaaagatacgaagaagttaaggctttcactgatacctacggtttcccaatcattattaaggctgcatttggtggtggtggtagaggtatgagagttgttagagatcaagcagaattgagagattctttcgaaagagctacttctgaagcaagatccgcttttggtaacggtaccgttttcgttgaaagatttttagacaagccaaagcatattgaagttcaattgttgggtgactcccatggtaacgttgttcacttgttcgaaagagactgttctgttcaaagaagacaccaaaaggttgttgaagttgctccagcaaaggatttgccagcagatgttagagacagaattttagctgacgctgttaagttggctaagtctgttaactacagaaacgcaggtactgctgaattcttggttgatcaacaaaacagacattacttcatcgaaattaacccaagaattcaagttgaacacactatcaccgaagaaatcactggtatcgatattgttgctgcacaaatccaaattgctgcaggtgcttccttggaacaattgggtttaacccaagacagaatttctgcaagaggtttcgctattcaatgtagaattactaccgaagacccagcaaagggtttttccccagatactggtaaaattgaagtttacagatctgctggtggtaacggtgttagattagatggtggtaacggtttcgctggtgcaattattaccccacattacgactccatgttggttaagtgtacttgtagaggttctacctacgaaattgcaagaagaaaggttgttagagctttggttgaattcagaatcagaggtgttaagactaacattccattcttgacctctttgttatcccacccaacttttgttgatggtaactgttggactaccttcattgatgacaccccagaattgttttctttagttggttcccaaaacagagcacaaaagttgttagcttacttaggtgacgttgctgttaacggttcttccattaagggtcaaattggtgaaccaaagttgaagggtgacgttattaagccaaagttattcgacgcagaaggtaaaccattggatgtttccgctccatgtaccaagggttggaagcaaattttagatagagaaggtccagctgcatttgctaaggcagttagagcaaacaagggttgtttgattatggacactacctggagagatgcacatcaatctttgttagctactagagttagaaccatcgatttgttgaacattgctcacgaaacttcttacgcatactccaacgcttactctttagaatgttggggtggtgcaaccttcgacgttgctatgagatttttatacgaagatccatgggacagattgagaaagatgagaaaggcagttccaaacattccattccaaatgttgttaagaggtgcaaacggtgttgcttactcttccttgccagataacgcaatctaccatttttgtaagcaagctaagaagtgtggtgttgacattttcagagttttcgatgctttgaacgatgttgaccaattggaagttggtattaaggcagttcatgctgcagaaggtgttgttgaagctactatgtgttactccggtgacatgttgaacccacacaagaagtacaacttagaatactacatggcattggttgataagattgttgctatgaagccacacattttaggtattaaggacatggcaggtgttttgaagccacaagctgcaagattgttggttggttctatcagacaaagatacccagacttgccaattcacgttcatactcacgattccgcaggtaccggtgttgcttctatgattgcttgtgcacaagctggtgcagatgctgttgacgctgcaactgattctatgtccggtatgacctctcaaccatccattggtgcaattttggcttccttagaaggtaccgaacaagatccaggtttgaacttagcacatgttagagctattgactcctactgggcacaattaagattgttatactctccattcgaagctggtttgactggtccagacccagaagtttacgaacacgaaattccaggtggtcaattgaccaacttaatcttccaagcttctcaattgggtttaggtcaacaatgggcagaaactaagaaggcttacgaagctgcaaacgacttgttaggtgacattgttaaggttactccaacctccaaggttgttggtgacttggcacaattcatggtttctaacaagttgaccccagaagacgttgttgaaagagctggtgaattagatttcccaggttccgttttggaatttttagaaggtttgatgggtcaaccattcggtggttttccagaaccattaagatctagagcattgagagatagaagaaagttggaaaagaggccaggtttgtacttagaaccattggacttagctaagattaagtcccaaatcagagaaaagttcggtgctgcaactgaatacgatgttgcatcttacgctatgtacccaaaggtttttgaagactacaagaagttcgttcaaaagtttggtgacttgtccgttttgccaaccagatacttcttagcaaagccagaaatcggtgaagaattccatgttgaattggaaaagggtaaagttttgatcttaaagttgttggctattggtccattgtctgaacaaactggtcaaagagaagttttctacgaagttaacggtgaagttagacaagttgcagttgatgacaacaaggcttccgttgataacacctctagaccaaaggcagatgttggtgactcttcccaagttggtgctccaatgtccggtgttgttgttgaaattagagttcatgacggtttagaagttaagaagggtgacccattagcagttttgtctgctatgaagatggaaatggttatttccgcaccacactctggtaaagtttcttccttgttagttaaggaaggtgactctgttgacggtcaagatttggtttgtaagattgttaaggcttaaatcactttctgtcaattgtcttaat

SEQ ID NO: 7 - DNA, 3599 bp, Pichia kudriavzevii
  misc_feature 1..3599: note = encoding PkPYC
  source 1..3599: mol_type = other DNA
caaaacacacaaacaaacacaattacaaaaaatgtcaactgtggaagatcactcctccttacataaattgagaaaggaatctgagattctttccaatgcaaacaaaatcttagtggctaatagaggtgaaattccaattagaattttcaggtcagcccatgaattgtcaatgcatactgtggcgatctattcccatgaagatcggttgtccatgcataggttgaaggccgacgaggcttatgcaatcggtaagacgggtcaatattcgccagttcaagcttatctacaaattgacgaaattatcaaaatagcaaaggaacatgatgtttccatgatccatccaggttatggtttcttatctgaaaactccgaattcgcaaagaaggttgaagaatccggtatgatttgggttgggcctcctgctgaagttattgattctgttggtgacaaggtttctgcaagaaatttggcaattaaatgtgacgttcctgttgttcctggtaccgatggtccaattgaagacattgaacaggctaaacagtttgtggaacaatatggttatcctgtcattataaaggctgcatttggtggtggtggtagaggtatgagagttgttagagaaggtgatgatatagttgatgctttccaaagagcgtcatctgaagcaaagtctgcctttggtaatggtacttgttttattgaaagatttttggataagccaaaacatattgaggttcaattattggctgataattatggtaacacaatccatctctttgaaagagattgttctgttcaaagaagacatcaaaaggttgttgaaattgcacctgccaaaactttacctgttgaagttagaaatgctatattaaaggatgctgtaacgttagctaaaaccgctaactatagaaatgctggtactgcagaatttttagttgattcccaaaacagacattattttattgaaattaatccaagaattcaagttgaacatacaattactgaagaaatcacaggtgttgatattgttgccgctcaaattcaaattgctgcaggtgcatcattggaacaattgggtctattacaaaacaaaattacaactagaggttttgcaattcaatgtagaattacaaccgaggatcctgctaagaattttgccccagatacaggtaaaattgaggtttatagatctgcaggtggtaatggtgtcagattagatggtggtaatgggtttgccggtgctgttatatctcctcattatgactcgatgttggttaaatgttcaacatctggttctaactatgaaattgccagaagaaagatgattagagctttagttgaatttagaatcagaggtgtcaagaccaatattcctttcttattggcattgctaactcatccagtcttcatttcgggtgattgttggacaacttttattgatgataccccttcgttattcgaaatggtttcttcaaagaatagagcccaaaaattattggcatatattggtgacttgtgtgtcaatggttcttcaattaaaggtcaaattggtttccctaaattgaacaaggaagcagaaatcccagatttgttggatccaaatgatgaggttattgatgtttctaaaccttctaccaatggtctaagaccatatctattaaagtatggaccagatgcattttccaaaaaagttcgtggattcgatggttgtatgattatggataccacctggagagatgcacatcaatcattattggctacaagagttagaactattgatttactgagaattgctccaacgactagtcatgccttacaaaatgcatttgcattagaatgttggggtggcgcaacatttgatgttgcgatgaggttcctctatgaagatccttgggagagattaagacaacttagaaaggcagttccaaatattcctttccaaatgttattgagaggtgctaatggtgttgcttattcgtcattacctgataatgcaattgatcattttgttaagcaagcaaaggataatggtgttgatattttcagagtctttgatgctttgaacgatttggaacaattgaaggttggtgttgatgctgtcaagaaagccggaggtgttgttgaagctacagtttgttactcaggtgatatgttaattccaggtaaaaagtataacttggattattatttagagactgttggaaagattgtggaaatgggtacccatattttaggtattaaggatatggctggcacgttaaagccaaaggctgctaagttgttgattggctcgatcagatcaaaataccctgacttggttatccatgtccatacccatgactctgctggtaccggtatttcaacttatgttgcatgcgcattggcaggtgccgacattgtcgattgtgcaatcaattcgatgtctggtttaacttctcaaccttcaatgagtgcttttattgctgctttagatggtgatatcgaaactggtgttccagaacattttgcaagacaattagatgcatattgggcagaaatgagattgttatactcatgtttcgaagccgacttgaagggaccagacccagaagtttataaacatgaaattccaggtggacagttgactaacctaatcttccaagcccaacaagttggtttgggtgaacaatgggaagaaactaagaagaagtatgaagatgctaacatgttgttgggtgatattgtcaaggttaccccaacctccaaggttgttggtgatttagcccaatttatggtttctaataaattagaaaaagaagatgttgaaaaacttgctaatgaattagatttcccagattcagttcttgatttctttgaaggattaatgggtacaccatatggtggattcccagagcctttgagaacaaatgtcatttccggcaagagaagaaaattaaagggtagaccaggtttagaattagaacctttcaacctcgaggaaatcagagaaaatttggtttccagatttggtccaggtattactgaatgtgatgttgcatcttataacatgtatccaaaggtttacgagcaatatcgtaaggtggttgaaaaatatggtgatttatctgttttaccaacaaaagcatttttggctcctccaactattggtgaagaagttcatgtggaaattgagcaaggtaagactttgattattaagttattagccatttctgacttgtctaaatctcatggtacaagagaagtatactttgaattgaatggtgaaatgagaaaggttacaattgaagataaaacagctgcaattgagactgttacaagagcaaaggctgacggacacaatccaaatgaagttggtgcgccaatggctggtgtcgttgttgaagttagagtgaagcatggaacagaagttaagaagggtgatccattagccgttttgagtgcaatgaaaatggaaatggttatttctgctcctgttagtggtagggtcggtgaagtttttgtcaacgaaggcgattccgttgatatgggtgatttgcttgtgaaaattgccaaagatgaagcgccagcagcttaaatcactttctgtcaattgtcttaat

SEQ ID NO: 8 - DNA, 1472 bp, synthetic construct
  misc_feature 1..1472: note = encoding PkFUM1
  source 1..1472: mol_type = other DNA
caaaacacacaaacaaacacaattacaaaaaatgttctcaactacctcaattgcaaaaagaatcgaaaaagatgcatttggtgacatcgaagtcccaaatgagaaatattggggtgctcaaactcaaagatctttacaaaatttcaaaattggtggtaagagagaagttatgccagaaccaatcatcaaatcttttggtattttaaagaaggctactgctaagatcaatgctgagtctggtgctttagacccaaagttatctgaagccattcaacaagctgcaaccgaagtttatgaaggtaaactaatggaccatttcccattagttgtctttcaaaccggttctggtactcaatctaacatgaatgccaatgaagtcatctctaatagagcaattgaaatcttgggtggtgaattaggctctaaaactccagtccatcctaatgatcatgttaatatgtcccaatcttctaatgatactttccctactgtcatgcatattgcagcagttacagaagtttcatcccatttattaccagaattgactgcactaagagatgcattgcaaaagaaatccgatgaatttaagaatattatcaaaatcggtagaacccatttacaagatgcaactcctttaactttaggtcaagaattttctggttatgttcaacaatgtactaatggtatcaaaagaatcgaaattgctcttgaacatttgagatacttagctcaaggtggtactgccgttggtactggtcttaacaccaagaaaggttttgctgaaaaggttgcaaatgaagtcaccaaattgaccggtttacaattctataccgctccaaataaattcgaagcccttgcagctcacgatgctgttgttgaaatgtctggtgctttgaataccgttgcagtctcattattcaaaatcgctcaagatatcagatatttgggttccggcccaagatgtggttatggtgaattggctttaccagaaaatgaaccaggttcttccatcatgccaggtaaagttaacccaactcaaaacgaagctttgactatgctttgtacccaagtctttggtaaccactcttgtattacctttgcaggtgcttcaggtcaattcgaattgaatgtctttaagccagttatgatctccaacttgttatcttctattaggttattaggtgatggttgtaattcttttagaatccactgtgttgaaggtatcattgcaaataccgacaagattgataaattactacatgaatctctcatgttagttactgctttgaacccacacattggttacgataaggcttccaagattgcaaagaatgcacacaagaagggcttgacattgaaacaatctgcattggaattaggttacttgaccgaagaacaattcaatgaatgggttagaccagaaaacatgattggtccaaaggattagatcactttctgtcaattgtcttaat

SEQ ID NO: 9 - protein, 239 aa, Pichia kudriavzevii
MTKETKKIIQVLSQYATCDMSDALVKHQYKLGGSLPNLHRYSANETKTTMVGKAYTVLFAPKDDPREAISGGYIDKLPEDSVLVIGTTLNLQKKDAPFTKMTNALYGGLMSTRANYLRSRGTVVFGRVRDIDEHLELKRDVFSYGLGTAAHGPVVKMVGINVPLEVLVDGYPEPHVETINPGDIIMGDDNGVVRVADSEELSSIMEYIPKRVQADTLVKEDILNGLECTPAQKKRRAGL

SEQ ID NO: 10 - protein, 575 aa, Pichia kudriavzevii
MTDKISLGTYLFEKLKEAGSYSIFGVPGDFNLALLDHVKEVEGIRWVGNANELNAGYEADGYARINGFASLITTFGVGELSAVNAIAGSYAEHVPLIHIVGMPSLSAMKNNLLLHHTLGDTRFDNFTEMSKKISAKVEIVYDLESAPKLINNLIETAYHTKRPVYLGLPSNFADELVPAALVKENKLHLEEPLNNPVAEEEFIHNVVEMVKKAEKPIILVDACAARHNISKEVRELAKLTKFPVFTTPMGKSTVDEDDEEFFGLYLGSLSAPDVKDIVGPTDCILSLGGLPSDFNTGSFSYGYTTKNVVEFHSNYCKFKSATYENLMMKGAVQRLISELKNIKYSNVSTLSPPKSKFAYESAKVAPEGIITQDYLWKRLSYFLKPRDIIVTETGTSSFGVLATHLPRDSKSISQVLWGSIGFSLPAAVGAAFAAEDAHKQTGEQERRTVLFIGDGSLQLTVQSISDAARWNIKPYIFILNNRGYTIEKLIHGRHEDYNQIQPWDHQLLLKLFADKTQYENHVVKSAKDLDALMKDEAFNKEDKIRVIELFLDEFDAPEILVAQAKLSDEINSKAA

SEQ ID NO: 11 - protein, 415 aa, Pichia kudriavzevii
MFLISKSLHFTRSFSNTIKTLNRSNIKMVSPAERLSTIASTIKPNRKDSTSLQPEDYPEHPFKVTVVGSGNWGCTIAKVIAENTVERPRQFQRDVNMWVYEELIEGEKLTEIINTKHENVKYLPGIKLPVNVVAVPDIVEACAGSDLIVFNIPHQFLPRILSQLKGKVNPKARAISCLKGLDVNPNGCKLLSTVITEELGIYCGALSGANLAPEVAQCKWSETTVAYTIPDDFRGKGKDIDHQILKSLFHRPYFHVRVISDVAGISIAGALKNVVAMAAGFVEGLGWGDNAKAAVMRIGLVETIQFAKTFFDGCHAATFTHESAGVADLITTCAGGRNVRVGRYMAQHSVSATEAEEKLLNGQSCQGIHTTREVYEFLSNMGRTDEFPLFTTTYRIIYENFPIEKLPECLEPVED

SEQ ID NO: 12 - protein, 350 aa, Pichia kudriavzevii
MSYEIPQTQKACVFYENGGPITYKDIPVPKPKPTEILVKVLYSGVCHTDLHAWKGDWPLATKLPLVGGHEGAGVVVAKGENVTSFEIGDYAGIKWLNGSCMGCEFCEQGAEPNCPKADLSGYTHDGSFQQYATADAIQAAHISKETDLAGVAPILCAGVTVYKALKTADLRAGEWVCISGAAGGLGSLAIQYAKAMGLRVVGIDGGDEKKELCKSLGAEAFIDFTKTKDIVKAVQEATNGGPHGVINVSVSEAAISQSCEYVRPLGKVVLVGLPAGAQVKTGVFEAVVKSIEIKGSYVGNRKDTAEALDFYTRGLVKSPFKIVGLSELPKVFELMEQGKILGRMVLDTSK

SEQ ID NO: 13 - protein, 262 aa, Pichia kudriavzevii
MASYKERSESHTSPVARRLFSIMEEKKSNLCASLDITETEKLLSILDTIGPYICLVKTHIDIVSDFTYEGTVLPLKELAKKHNFMIFEDRKFADIGNTVKNQYKSGVFRIAEWADITNAHGVTGAGIVSGLKEAAQETTSEPRGLLMLAELSSKGSLAYGEYTEKTVEIAKSDKEFVIGFIAQHDMGGREEGFDWIIMTPGVGLDDKGDALGQQYRTVDEVVKTGTDIIIVGRGLYGQGRDPVEQAKRYQQAGWNAYLNRFK

SEQ ID NO: 14 - protein, 539 aa, Pichia kudriavzevii
MTLHKNSNEGVQASGFELQDNLDVPHSNASFQSFKSDEAEQAHNNEHLMEKPQFNKATISNYCKTRFTELFPTKQSMAANKHLLNPLPGLRMIGFKQWLLILSGFLAWTWDAYDFFSISLNTVQLAKDFDKTVKDITWGITVVLMLRSVGGFFFGYLGDKYGRKWPLIANLMCVCFLEIGTGFIKNYSQFLGVRAVFGIMLGGVYGNAAATALDDCPAEARGFISGFLQQGYAFGYLLAVVFKRAIADNSPHRWRAMFWFGAGVCFLICCFRAVLPETKAFQRNKEIERYNEEHGIHQRSFKEKATTSLKIYWLMIIYMVLLMAGFNFMSHGSQDLYPTLLTVRYNFSDNATTVTNCVANIGAITGGIIIGHFSNFIGRRLSIIICCIIGGALIYPWAFVDNANINAGAFFLQFFVQGAWGVVPVHLSELAPPDFKAFVVGIAYQLGNLASSASSTIETTIGVHFPMTSPGGEPIFDYAKVMAIFVGCVFAYVLLITFIGPERKSVSFEEPVDEDIEINEKIKHNEEIEAGSNLGTSRA

SEQ ID NO: 15 - protein, 523 aa, Pichia kudriavzevii
MSDLESQHTREELDKSEDEEIQLINESRPPKLDKETIKRYLKTRFTELLPTKQQMKQNKHLLNPLPGLRMMGRRQWLMFLSAFCAWTWDAYDFFTVSLNTVQLAKDFDKNVKDITWGITLVLMLRSVGGITFGYLGDRYGRKWPLVANLLIVCILEIGSGFIKTYRQFLGVRALFGICLGGVYGNATATALDDCPTEARGFIGGLLQQGYAFGYLLAVVFKRAIADNSSHKWRATFWFGAGISFLFALFRASLPETKAFLRKKEIERYNKEHGIYQPTFQMKIVESLKNYWLMMIYLVLFMSGFSFMSHSSQDLYPTLLTVRYSFSENKATVTNCVANIGAFIGGVFTGHISNFLGRRLTIMLICIFGGALIYPWAFIDGTGINAGVFFLQWCVQGGLGVVPSHLSELAPPDLRAFVVGISYQLGNLAASASSTIETTIGEQFPMTSPSGEPIYDYAKVMAIFVGCVFAFVLIVTLFGPERRNASFENAVTTNEEFGNSAGAVDKIEHVEECIVPKHARNQQC

SEQ ID NO: 16 - protein, 506 aa, Pichia kudriavzevii
MFNPSIGEVDPSRRSSIVTAEVAKAHIKSNQRNGPEDHLHTSNDYVGYEFELSHLRTNPNNNQTINGKVQEYNVSTIEENSEDEDHDDSVYPNGYAPLLVVFGGFLSCFTLFGIMNSVGAIESYIQVNQLANASVTAISWVFSIYMFITLFSGLIVGPLYDTFGATYLMIIGTLFTFTGLLACGSSKDIYQFVLSFGVCTGIGSGCLMFPSISVISSWFNRTKRSFYIGLIQTGGSVGGVCFPILLRYLYAKYGFVWAMRIFAFFNLGVCSVACIFVRDRINEIRELTNEPIDDRTFWEKFKNSFDIRSFKDKKFIVLTAALFMNEFSLLIVITYLASYAIANGASISESYVMITIMNVSGTFGKFIPSYFAQRYGCFNMMIIMSVSMTIECFVIWLPFGKHKGALYLFIVLFGFAYAATYSLTGATIGAITPKTKDFGKRYGSAYAIVSFGNLISLPISGAFIVNRTASDYDNMVAFAASTCALASVLFLFSRYTIVGRKLRCKI

SEQ ID NO: 17 - DNA, 601 bp, Pichia kudriavzevii
  source 1..601: mol_type = other DNA
cgatgccatattgtatgtgtattgtattaagtgtgtattgtcttaagtgtgtaagagacatttatttgtgtcaacaatagcgacgccactgaaaacctcaaatatcgtatttattaatccccttcccccaagcgcagatcgtcccgtcgatttctattgtttgggcattatcagcgacgcgacggcgacgcgacggcgataatgggcgacggtcacaagatggaacgagaaaacagtttttttcggataggactcattttccaggtgagaatggggtgaccccggggagaaaccttccgcgagtggagtgcgagtggagtgggaaatgtggcccccccccccttgtgggccatgaggttgacaaataccgtgtggcccggtgatggagtgagaaagagagggaaatgataatgggaaaacaaggagaggcccgtttcccgggatttatataaagaggtgtctctatcccagttgaagtagagatttgttgatgtagttgttccttccaataaatttgttcaatcagtacacagctaatactattattacagctactactaatactactactactattactaccacccccaacacaaacaca

SEQ ID NO: 18 - DNA, 513 bp, Pichia kudriavzevii
  source 1..513: mol_type = other DNA
ctacaacaagatgtttgttcaaggggagcaacttgtccctcgttaaataatttgtaagaaaaaacttcttccttttatctctttccttttttttttttaaaaaaactatctagtaaggaaatatacacaatttactttgtacgctgtctctctttctctatctctctctatgtctatctctccctatcgctctgtatgtatgtacattaccgtcttccccaaatggctcaacccgactgcgagaagacttcaaaacactcaattatggtctttagattttccagtacgttgttgacagataccctcactattctgtcgtcgacccccctcaccgagatgttcaattgagagtcttgcacagaatactccaacgaggactggtcagacttgaggacagggtctggtctgagagcatcacgagcaattcttgcctgttcaatagatccaaaggggatattgacctgcaccgatacggggaatggcatggattggtgggatggtatggtaatcttc

SEQ ID NO: 19 - DNA, 865 bp, Pichia kudriavzevii
  source 1..865: mol_type = other DNA
cctgttggcgtatctacatcacttcctacaaacaacaccacgaattgcgtccgtggtgacgcaactacgaatggcattgtcaatgccaatgccagtgcacatacacgtgcaagtcccaccggttccctgcccggctatggtagagacaagaaggacgataccggcatcgacatcaacagtttcaacagcaatgcgtttggcgtcgacgcgtcgatggggctgccgtatttggatttggacgggctagatttcgatatggatatggatatggatatggagatgaatttgaatttagatttgggtcttgatttggggttggaattaaaaggggataacaatgagggttttcctgttgatttaaacaatggacgtgggaggtgattgatttaacctgatccaaaaggggtatgtctattttttagagtgtgtctttgtgtcaaattatggtagaatgtgtaaagtagtataaactttcctctcaaatgacgaggtttaaaacaccccccgggtgagccgagccgagaatggggcaattgttcaatgtgaaatagaagtatcgagtgagaaacttgggtgttggccagccaaggggggggggggaaggaaaatggcgcgaatgctcaggtgagattgttttggaattgggtgaagcgaggaaatgagcgacccggaggttgtgactttagtggcggaggaggacggaggaaaagccaagagggaagtgtatataaggggagcaatttgccaccaggatagaattggatgagttataattctactgtatttattgtataatttatttctccttttatatcaaacacattacaaaacacacaaaacacacaaacaaacacaattacaaaaa

SEQ ID NO: 20 - DNA, 481 bp, Pichia kudriavzevii
  source 1..481: mol_type = other DNA
atcactttctgtcaattgtcttaattattttaatatggtatttttatttgaaatactaaagcacattttcctttccacatttaatttcttaatgaactttatttctttatgatttctagatctatatttctatttgtcaactaactagattaattttaacacttacatttcttttttaaaactatgaatcataacatgcttgatagctcttatttgttttttttttacagatcaaaaaacaccttttgtagaagtaattggtctggtttgtatgtgacattaatactattttctttggaaggccgtatacatggaactaaatattttacctaacacataaaattttatttttccaaccaaagaaaaggctgaaacggatattttcttcacgttatcgaaaaataaaagcctagttaaaattgataatgaatcctgaaacgtaatcataaatagtttagaatactagctaaatcggtatcgc

SEQ ID NO: 21 - DNA, 507 bp, Pichia kudriavzevii
  source 1..507: mol_type = other DNA
gcagcctctacgttgagaataatgttcccacccccgggcgagacttctgcgggggggcatgagtgcgggaaacgccggagtccgttcggtggtattgttttacattttcgttattacccaacgggggctattggtcttcaatgaggaagttctggaaattgtcggatagaaaatagtcccaattctattgttactaatggcgctagtgatattgttgcagtaaatggtcaattcccaattattccatacacggggtgcgtcggcgcgagggtagggtgatggttttcacctttggtgggcctcaatgtgagggtgggtggcatcatagtcaagataacaaattgtacaccaactcttataaaaggacacccatttgccgccatgtatattggttgatgtgtatttgttatttttccaattatattattttgtctttgatttttttattttagtttcttttaacatcaattaaatccaaacgaaccccccctccccctattagaaaaa

SEQ ID NO: 22 - DNA, 531 bp, Pichia kudriavzevii
  source 1..531: mol_type = other DNA
gtctagagagtgtatacctccccgcttttgctgctactaattaatacccactattaatttccttctattacaaaacgcctctcagactcccacacacacacttacatatgtacacgctcatacatacacttataaacatacatatatacgtcgacgatataattttaatgtcaatagtcatgaacatttgaactactttcccgtttctctattttccggtttctttcccaaccgtcttttgtctttctttccacgtggctgacccaacgttttccattcacagagtgcattgtctattgtggaaaagcgggggtgagatttccacaaaacctgtacttctcacctcccccctccttaaccccggcccaaggggggggggtacgcggcactgtagttaaggccgtacggagattttcccgggtgtcggcgtttagagacacacacaatagagagttttacttggaatacaatacacccccactctaattgtgtgttcatctcttctcctttcctctccgcttgtctcaagag

SEQ ID NO: 23 - DNA, 9052 bp, synthetic construct
  misc_feature 1..9052: note = pWSPK_backbone
  source 1..9052: mol_type = other DNA
cttaccagaataatatgcagtttgctataaaaggaacaatagatctcaccggtacgaaccgccaatcaaattcccacagcgtgatatccttttcagaagacaaaaggagcaatataaaaaatgctacattgtgttatgcctaatgggatagaaaatataactctttccattactcttctggtttttattggaacaatcactcttgcaaatttccttgactgccacgttatgaatgaagaacaattacactgagggattttaaagctgccctgtagagtgatgtccttttgttaaagtctgttacactacaacaatggttttgaaaaaaaaaacccattgagaaattaaccaaagtccgggattatcggaagagcgcaacttaataaacacatcgttacaaaatatttttttttcattaaattcatttataaacgtagggactgtaaaaattgtactagatatttagtaaaagcattagttagattcatttaaatctgtttaaataagcattccaaccagcttgttggtatcttttagcttgctctataggatctcttccttgaccgtacaaacctctaccaacaattatgatatccgttccagtctttacaacttcatcaacagttctatattgttgaccaagtgcatcacctttgtcatctaaaccaacccctggagtcataatgatccagtcaaaaccttcttctctaccgcccatatcgtgttgcgcaataaaaccaatgacaaactctttatcagatttagcaatttctactgttttttctgtatattcaccatatgctaaagaaccctttgatgataactcagcaagcattagcaaacctctaggttcactggttgtttcttgggctgcctccttcaagccagaaacaatacctgcacctgttacaccatgtgcattagtgatgtcagcccattcggcaatacggaagacaccagatttatattgatttttaacagtgttaccaatatcagcaaattttctatcttcaaaaatcataaaattatgtttcttggcaagctccttcaaaggcaacacagttccttcatacgtaaaatcagaaacaatatcgatgtgtgttttaactagacagatgtaaggaccaatagtgtccaaaatagagagaagcttttcagtttcagtaatatccaatgatgcacaaaggttagacttcttttcctccatgatggagaaaagtctcctagcaacaggggaagtgtgtgattctgatctttctttgtatgacgccatccttgacaaacaaactactttattaaagcgttgaagatctattctccagcaattaaatttgtgaagaataactggtatagagtacttcctttaaaaacatgtccgtgcaccaagaaaaaaaaaaagtttgaaaaattgtatgtcgacgaatttcagcattttcatttcaaggcgatattatgtttcactaaactcaggacaggaatatactaagaataactacaacatacacacaacataagccaagatggatcaacttaactaccaagaacaacaacaatttcaaaagatcgttgaacaaaagcaaatggctgatttcatgaggctatacacatctcttgtggacagatgtttcaacgattgtgttcaagacttcacctctgaatccttaaccagcagagaaagttcatgtctaaccaaatgtgctgaaaaatttttgaagcactctgagagagttggtacccgtttccaagaacagaaccaaaagttaatgaaccaaatgagacaatgattgccgctagacaatgtcaaccttccctgtttctcgagacgcaaaccgcctctccccgcgcgttggccgattcattaatgcagctggcacgacaggtttcccgactggaaagcgggcagtgagcgcaacgcaattaatgtgagttagctcactcattaggcaccccaggctttacactttatgcttccggctcgtatgttgtgtggaattgtgagcggataacaatttcacacaggaaacagctatgaccatgattacgccaagcttgcatgcctgcaggtcgactctagaggatcctctaatggtgtacacttgaacctggttggcccattatcacttctacaagtctggaaagaatagcctatttggttcatcttcggatccccgggtaccgagctcgaattcactggccgtcgttttacaacgtcgtgactgggaaaaccctggcgttacccaacggggggcccggtacccaattcgccctatagtgagtcgtattacgcgcgcaagaatacaacaaaagaatttgtgtttctacagatgttttcggtagaggtattgatatcgaaagaatcaacttggccatcaactacgatatgccaagtgaagcagatcagtacttgcacagagttggtagagcaggtagattcggtactaaaggtttggctgtttcctttatctctaatgaaaaggatgaagaaatcttgaacaagatccaagataggtttgatgttaagattcaagagttccctgaagaaggtgttgatccttctacttacatgaacacttaattgacattgatctgtcatagttttgtggttgttttttttttgaagttatatacatttattaatatatctttatatatatattgtccaaatccatcggaaagggtctactgtaatacaatcccatatagtagaatgtactcttatatgctgcaatgaggacttgctctggagatatcgttgataagggactaccttggcttccaacgcgttggtcaacaaactgaccttgaagtgcaaatcccgacaggcacgcgtgagatatcggaggtgaatgcacctccaaatcagacaacgcgagcaaacgacgcgtaacacaaggcttgacgcgtacgatgcagacttttcatagtgtgtcgccactgagcgggaggcgggttataaaagaaacgtgtttggcgtatcttttctcttctctggatttgttcttctacttcctttactcctcatcaaatcgtctctccctcgtcactcaccacaactagtccgacactatctgatatacccttattgctaactatggacaagaagtactccattgggctcgatatcggcacaaacagcgtcggttgggccgtcattacggacgagtacaaggtgccgagcaaaaaattcaaagttctgggcaataccgatcgccacagcataaagaagaacctcattggcgccctcctgttcgactccggggagacggccgaagccacgcggctcaaaagaacagcacggcgcagatatacccgcagaaagaatcggatctgctacctgcaggagatctttagtaatgagatggctaaggtggatgactctttcttccataggctggaggagtcctttttggtggaggaggataaaaagcacgagcgccacccaatctttggcaatatcgtggacgaggtggcgtaccatgaaaagtacccaaccatatatcatctgaggaagaagcttgtagacagtactgataaggctgacttgcggttgatctatctcgcgctggcgcatatgatcaaatttcggggacacttcctcatcgagggggacctgaacccagacaacagcgatgtcgacaaactctttatccaactggttcagacttacaatcagcttttcgaagagaacccgatcaacgcatccggagttgacgccaaagcaatcctgagcgctaggctgtccaaatcccggcggctcgaaaacctcatcgcacagctccctggggagaagaagaacggcctgtttggtaatcttatcgccctgtcactcgggctgacccccaactttaaatctaacttcgacctggccgaagatgccaagcttcaactgagcaaagacacctacgatgatgatctcgacaatctgctggcccagatcggcgaccagtacgcagacctttttttggcggcaaagaacctgtcagacgccattctgctgagtgatattctgcgagtgaacacggagatcaccaaagctccgctgagcgctagtatgatcaagcgctatgatgagcaccaccaagacttgactttgctgaaggcccttgtcagacagcaactgcctgagaagtacaaggaaattttcttcgatcagtctaaaaatggctacgccggatacattgacggcggagcaagccaggaggaattttacaaatttattaagcccatcttggaaaaaatggacggcaccgaggagctgctggtaaagcttaacagagaagatctgttgcgcaaacagcgcactttcgacaatggaagcatcccccaccagattcacctgggcgaactgcacgctatcctcaggcggcaagaggatttctacccctttttgaaagataacagggaaaagattgagaaaatcctcacatttcggataccctactatgtaggccccctcgcccggggaaattccagattcgcgtggatgactcgcaaatcagaagagaccatcactccctggaacttcgaggaagtcgtggataagggggcctctgcccagtccttcatcgaaaggatgactaactttgataaaaatctgcctaacgaaaaggtgcttcctaaacactctctgctgtacgagtacttcacagtttataacgagctcaccaaggtcaaatacgtcacagaagggatgagaaagccagcattcctgtctggagagcagaagaaagctatcgtggacctcctcttcaagacgaaccggaaagttaccgtgaaacagctcaaagaagactatttcaaaaagattgaatgtttcgactctgttgaaatcagcggagtggaggatcgcttcaacgcatccctgggaacgtatcacgatctcctgaaaatcattaaagacaaggacttcctggacaatgaggagaacgaggacattcttgaggacattgtcctcacccttacgttgtttgaagatagggagatgattgaagaacgcttgaaaacttacgctcatctcttcgacgacaaagtcatgaaacagctcaagaggcgccgatatacaggatgggggcggctgtcaagaaaactgatcaatgggatccgagacaagcagagtggaaagacaatcctggattttcttaagtccgatggatttgccaaccggaacttcatgcagttgatccatgatgactctctcacctttaaggaggacatccagaaagcacaagtttctggccagggggacagtcttcacgagcacatcgctaatcttgcaggtagcccagctatcaaaaagggaatactgcagaccgttaaggtcgtggatgaactcgtcaaagtaatgggaaggcataagcccgagaatatcgttatcgagatggcccgagagaaccaaactacccagaagggacagaagaacagtagggaaaggatgaagaggattgaagagggtataaaagaactggggtcccaaatccttaaggaacacccagttgaaaacacccagcttcagaatgagaagctctacctgtactacctgcagaacggcagggacatgtacgtggatcaggaactggacatcaatcggctctccgactacgacgtggatcatatcgtgccccagtcttttctcaaagatgattctattgataataaagtgttgacaagatccgataaaaatagagggaagagtgataacgtcccctcagaagaagttgtcaagaaaatgaaaaattattggcggcagctgctgaacgccaaactgatcacacaacggaagttcgataatctgactaaggctgaacgaggtggcctgtctgagttggataaagccggcttcatcaaaaggcagcttgttgagacacgccagatcaccaagcacgtggcccaaattctcgattcacgcatgaacaccaagtacgatgaaaatgacaaactgattcgagaggtgaaagttattactctgaagtctaagctggtctcagatttcagaaaggactttcagttttataaggtgagagagatcaacaattaccaccatgcgcatgatgcctacctgaatgcagtggtaggcactgcacttatcaaaaaatatcccaagcttgaatctgaatttgtttacggagactataaagtgtacgatgttaggaaaatgatcgcaaagtctgagcaggaaataggcaaggccaccgctaagtacttcttttacagcaatattatgaattttttcaagaccgagattacactggccaatggagagattcggaagcgaccacttatcgaaacaaacggagaaacaggagaaatcgtgtgggacaagggtagggatttcgcgacagtccggaaggtcctgtccatgccgcaggtgaacatcgttaaaaagaccgaagtacagaccggaggcttctccaaggaaagtatcctcccgaaaaggaacagcgacaagctgatcgcacgcaaaaaagattgggaccccaagaaatacggcggattcgattctcctacagtcgcttacagtgtactggttgtggccaaagtggagaaagggaagtctaaaaaactcaaaagcgtcaaggaactgctgggcatcacaatcatggagcgatcaagcttcgaaaaaaaccccatcgactttctcgaggcgaaaggatataaagaggtcaaaaaagacctcatcattaagcttcccaagtactctctctttgagcttgaaaacggccggaaacgaatgctcgctagtgcgggcgagctgcagaaaggtaacgagctggcactgccctctaaatacgttaatttcttgtatctggccagccactatgaaaagctcaaagggtctcccgaagataatgagcagaagcagctgttcgtggaacaacacaaacactaccttgatgagatcatcgagcaaataagcgaattctccaaaagagtgatcctcgccgacgctaacctcgataaggtgctttctgcttacaataagcacagggataagcccatcagggagcaggcagaaaacattatccacttgtttactctgaccaacttgggcgcgcctgcagccttcaagtacttcgacaccaccatagacagaaagcggtacacctctacaaaggaggtcctggacgccacactgattcatcagtcaattacggggctctatgaaacaagaatcgacctctctcagctcggtggagacagcagggctgaccccaagaagaagaggaaggtgtgagtgagctgatagtttcttcttttacccttatatttattaaaatactcttaataatatcccatcttacatataacgaattccattcttgtcttatattcttaatcatgtcctagaaatcaaacaaaaaaaaatgtttataatgatttttttagtgttttatacattttctgtatagaagaaaaaaaaagactattattatacttacattgtaacacaattgcaacgagtgtaatttttaggttttcgttttccccctcacagctcgattattgtcaaatcacacgacaagaaaacgtaaaagcaaaaggccaggaaccgtaaaaaggccgcgttgctggcgtttttccataggctccgcccccctgacgagcatcacaaaaatcgacgctcaagtcagaggtggcgaaacccgacaggactataaagataccaggcgtttccccctggaagctccctcgtgcgctctcctgttccgaccctgccgcttaccggatacctgtccgcctttctcccttcgggaagcgtggcgctttctcatagctcacgctgtaggtatctcagttcggtgtaggtcgttcgctccaagctgggctgtgtgcacgaaccccccgttcagcccgaccgctgcgccttatccggtaactatcgtcttgagtccaacccggtaagacacgacttatcgccactggcagcagccactggtaacaggattagcagagcgaggtatgtaggcggtgctacagagttcttgaagtggtggcctaactacggctacactagaagaacagtatttggtatctgcgctctgctgaagccagttaccttcggaaaaagagttggtagctcttgatccggcaaacaaaccaccgctggtagcggtggtttttttgtttgcaagcagcagattacgcgcagaaaaaaaggatctcaagaagatcctttgatcttttctacggggtctgacgctcagtggaacgaaaactcacgttaagggattttggtcatgagattatcaaaaaggatcttcacctagatccttttaaattaaaaatgaagttttaaatcaatctaaagtatatatgagtaaacttggtctgacagttaccaatgcttaatcagtgaggcacctatctcagcgatctgtctatttcgttcatccatagttgcctgactccccgtcgtgtagataactacgatacgggagggcttaccatctggccccagtgctgcaatgataccgcgagacccacgctcaccggctccagatttatcagcaataaaccagccagccggaagggccgagcgcagaagtggtcctgcaactttatccgcctccatccagtctattaattgttgccgggaagctagagtaagtagttcgccagttaatagtttgcgcaacgttgttgccattgctacaggcatcgtggtgtcacgctcgtcgtttggtatggcttcattcagctccggttcccaacgatcaaggcgagttacatgatcccccatgttgtgcaaaaaagcggttagctccttcggtcctccgatcgttgtcagaagtaagttggccgcagtgttatcactcatggttatggcagcactgcataattctcttactgtcatgccatccgtaagatgcttttctgtgactggtgagtactcaaccaagtcattctgagaatagtgtatgcggcgaccgagttgctcttgcccggcgtcaatacgggataataccgcgccacatagcagaactttaaaagtgctcatcattggaaaacgttcttcggggcgaaaactctcaaggatcttaccgctgttgagatc

SEQ ID NO: 24 - DNA, 26 bp, synthetic construct
  misc_feature 1..26: note = 1_UP_2365_F
  source 1..26: mol_type = other DNA
ggtgtccactcatatacttcattttc

SEQ ID NO: 25 - DNA, 50 bp, synthetic construct
  misc_feature 1..50: note = 1_UP_2365_R1
  source 1..50: mol_type = other DNA
acaatacacatacaatatggcatcgctgaatactatcgaatcttgccaac

SEQ ID NO: 26 - DNA, 25 bp, synthetic construct
  misc_feature 1..25: note = 1_UP_2365_R2
  source 1..25: mol_type = other DNA
ctgaatactatcgaatcttgccaac

SEQ ID NO: 27 - DNA, 25 bp, synthetic construct
  misc_feature 1..25: note = 2_PFBA1_F
  source 1..25: mol_type = other DNA
cgatgccatattgtatgtgtattgt

SEQ ID NO: 28 - DNA, 23 bp, synthetic construct
  misc_feature 1..23: note = 2_PFBA1_R
  source 1..23: mol_type = other DNA
tgtgtttgtgttgggggtggtag

SEQ ID NO: 29 - DNA, 49 bp, synthetic construct
  misc_feature 1..49: note = 3_SbMDH_F
  source 1..49: mol_type = other DNA
actaccacccccaacacaaacacaatgggtttgtctaccgcatactctc

SEQ ID NO: 30 - DNA, 49 bp, synthetic construct
  misc_feature 1..49: note = 3_SbMDH_R
  source 1..49: mol_type = other DNA
cccttgaacaaacatcttgttgtagttaaacttcacctggcaacatagt

SEQ ID NO: 31 - DNA, 24 bp, synthetic construct
  misc_feature 1..24: note = 4_TINO1_F
  source 1..24: mol_type = other DNA
ctacaacaagatgtttgttcaagg

SEQ ID NO: 32 - DNA, 23 bp, synthetic construct
  misc_feature 1..23: note = 4_TINO1_R
  source 1..23: mol_type = other DNA
gaagattaccataccatcccacc

SEQ ID NO: 33 - DNA, 52 bp, synthetic construct
  misc_feature 1..52: note = 5_DW_2365_F1
  source 1..52: mol_type = other DNA
gattggtgggatggtatggtaatcttcgatgagcatctagagttgaagaggg

SEQ ID NO: 34 - DNA, 50 bp, synthetic construct
  misc_feature 1..50: note = 5_DW_2365_F2
  source 1..50: mol_type = other DNA
gttggcaagattcgatagtattcaggatgagcatctagagttgaagaggg

SEQ ID NO: 35 - DNA, 24 bp, synthetic construct
  misc_feature 1..24: note = 5_DW_2365_R
  source 1..24: mol_type = other DNA
ccgacttgtacgaatttgttcctc

SEQ ID NO: 36 - DNA, 26 bp, synthetic construct
  misc_feature 1..26: note = pWSPK-F
  source 1..26: mol_type = other DNA
cttaccagaataatatgcagtttgct

SEQ ID NO: 37 - DNA, 25 bp, synthetic construct
  misc_feature 1..25: note = pWSPK-R
  source 1..25: mol_type = other DNA
gatctcaacagcggtaagatccttg

SEQ ID NO: 38 - DNA, 25 bp, synthetic construct
  misc_feature 1..25: note = sgRNA-1F
  source 1..25: mol_type = other DNA
caaggatcttaccgctgttgagatc

SEQ ID NO: 39 - DNA, 65 bp, synthetic construct
  misc_feature 1..65: note = 2365_sgRNA-1R
  source 1..65: mol_type = other DNA
aacttgctatttctagctctaaaacctctcggatcatcctttggctgcgcaagcccggaatcgaa

SEQ ID NO: 40 - DNA, 34 bp, synthetic construct
  misc_feature 1..34: note = sgRNA-2F
  source 1..34: mol_type = other DNA
gttttagagctagaaatagcaagttaaaataagg

SEQ ID NO: 41 - DNA, 26 bp, synthetic construct
  misc_feature 1..26: note = sgRNA-2R
  source 1..26: mol_type = other DNA
agcaaactgcatattattctggtaag

SEQ ID NO: 42 - DNA, 28 bp, synthetic construct
  misc_feature 1..28: note = 1_PADH1_F
  source 1..28: mol_type = other DNA
gcagcctctacgttgagaataatgttcc

SEQ ID NO: 43 - DNA, 26 bp, synthetic construct
  misc_feature 1..26: note = 1_PADH1_R
  source 1..26: mol_type = other DNA
tttttctaatagggggagggggggtt

SEQ ID NO: 44 - DNA, 50 bp, synthetic construct
  misc_feature 1..50: note = 2_ScFRD_F
  source 1..50: mol_type = other DNA
accccccctccccctattagaaaaaatgtccttgtctccagttgttgtta

SEQ ID NO: 45 - DNA, 58 bp, synthetic construct
  misc_feature 1..58: note = 2_ScFRD_R
  source 1..58: mol_type = other DNA
aaagcggggaggtatacactctctagacttactttctatcgttagcaatagattcagc

SEQ ID NO: 46 - DNA, 48 bp, synthetic construct
  misc_feature 1..48: note = 2_LmFRD_F
  source 1..48: mol_type = other DNA
accccccctccccctattagaaaaaatggctgatggtaaaacttctgc

SEQ ID NO: 47 - DNA, 52 bp, synthetic construct
  misc_feature 1..52: note = 2_LmFRD_R
  source 1..52: mol_type = other DNA
aaagcggggaggtatacactctctagacttaggatggtggttcggtttcgtc

SEQ ID NO: 48 - DNA, 49 bp, synthetic construct
  misc_feature 1..49: note = 2_TbFRD_F
  source 1..49: mol_type = other DNA
accccccctccccctattagaaaaaatggttgatggtagatcttccgca

SEQ ID NO: 49 - DNA, 52 bp, synthetic construct
  misc_feature 1..52: note = 2_TbFRD_R
  source 1..52: mol_type = other DNA
aaagcggggaggtatacactctctagacttaggaaccagatggttcggtttc

SEQ ID NO: 50 - DNA, 27 bp, synthetic construct
  misc_feature 1..27: note = 3_TADH1_F1
  source 1..27: mol_type = other DNA
gtctagagagtgtatacctccccgctt

SEQ ID NO: 51 - DNA, 52 bp, synthetic construct
  misc_feature 1..52: note = 3_TADH1_F2
  source 1..52: mol_type = other DNA
accccccctccccctattagaaaaagtctagagagtgtatacctccccgctt

SEQ ID NO: 52 - DNA, 25 bp, synthetic construct
  misc_feature 1..25: note = 3_TADH1_R
  source 1..25: mol_type = other DNA
ctcttgagacaagcggagaggaaag

SEQ ID NO: 53 - DNA, 65 bp, synthetic construct
  misc_feature 1..65: note = ADH1_sgRNA-1R
  source 1..65: mol_type = other DNA
aacttgctatttctagctctaaaacgctctaaggtctgcagtctttgcgcaagcccggaatcgaa

SEQ ID NO: 54 - DNA, 28 bp, synthetic construct
  misc_feature 1..28: note = PDC1_1F
  source 1..28: mol_type = other DNA
ccgtatcttattgtatcctatcctattc

SEQ ID NO: 55 - DNA, 54 bp, synthetic construct
  misc_feature 1..54: note = PDC1_1R
  source 1..54: mol_type = other DNA
atgttcattttacattcagatgtcaatttttatgttttgctgtgttttgtttta

SEQ ID NO: 56 - DNA, 39 bp, synthetic construct
  misc_feature 1..39: note = PDC1_2F
  source 1..39: mol_type = other DNA
acataaaaattgacatctgaatgtaaaatgaacattaaa

SEQ ID NO: 57 - DNA, 24 bp, synthetic construct
  misc_feature 1..24: note = PDC1_2R
  source 1..24: mol_type = other DNA
gttgaagtcaacgaagatggtgag

SEQ ID NO: 58 - DNA, 65 bp, synthetic construct
  misc_feature 1..65: note = PDC1_sgRNA-1R
  source 1..65: mol_type = other DNA
aacttgctatttctagctctaaaacgcattcaactcgttagcgtttgcgcaagcccggaatcgaa

SEQ ID NO: 59 - DNA, 27 bp, synthetic construct
  misc_feature 1..27: note = GPD1_1F
  source 1..27: mol_type = other DNA
ctctacaagagaggaaacacactacag

SEQ ID NO: 60 - DNA, 34 bp, synthetic construct
  misc_feature 1..34: note = GPD1_1R
  source 1..34: mol_type = other DNA
aaaataaatttaaaataaacgatatcaaaattca

SEQ ID NO: 61 - DNA, 59 bp, synthetic construct
  misc_feature 1..59: note = GPD1_2F
  source 1..59: mol_type = other DNA
gaattttgatatcgtttattttaaatttattttataacctcaaggagaactttggcatt

SEQ ID NO: 62 - DNA, 27 bp, synthetic construct
  misc_feature 1..27: note = GPD1_2R
  source 1..27: mol_type = other DNA
gaaatctatgcaaaccactctctcctg

SEQ ID NO: 63 - DNA, 65 bp, synthetic construct
  misc_feature 1..65: note = GPD1_sgRNA-1R
  source 1..65: mol_type = other DNA
aacttgctatttctagctctaaaacgcagattcatgagtaaaggttgcgcaagcccggaatcgaa

SEQ ID NO: 64 - DNA, 25 bp, synthetic construct
  misc_feature 1..25: note = 1_UP_MCH4_F
  source 1..25: mol_type = other DNA
aactttgttgtacattaagcgagtg

SEQ ID NO: 65 - DNA, 47 bp, synthetic construct
  misc_feature 1..47: note = 1_UP_MCH4_R1
  source 1..47: mol_type = other DNA
gaagtgatgtagatacgccaacaggagcagttgataatggaaaggga

SEQ ID NO: 66 - DNA, 26 bp, synthetic construct
  misc_feature 1..26: note = 1_UP_MCH4_R2
  source 1..26: mol_type = other DNA
agcagttgataatggaaagggatagg

SEQ ID NO: 67 - DNA, 25 bp, synthetic construct
  misc_feature 1..25: note = 2_PTDH3_F
  source 1..25: mol_type = other DNA
cctgttggcgtatctacatcacttc

SEQ ID NO: 68 - DNA, 31 bp, synthetic construct
  misc_feature 1..31: note = 2_PTDH3_R
  source 1..31: mol_type = other DNA
tttttgtaattgtgtttgtttgtgtgttttg

SEQ ID NO: 69 - DNA, 59 bp, synthetic construct
  misc_feature 1..59: note = 3_SpMAE1_F
  source 1..59: mol_type = other DNA
caaaacacacaaacaaacacaattacaaaaaatgggtgaattaaaggaaatcttaaagc

SEQ ID NO: 70 - DNA, 49 bp, synthetic construct
  misc_feature 1..49: note = 3_SpMAE1_R
  source 1..49: mol_type = other DNA
attaagacaattgacagaaagtgatttagacggattcgtgttcagagga

SEQ ID NO: 71 - DNA, 25 bp, synthetic construct
  misc_feature 1..25: note = 4_TGAL2_F
  source 1..25: mol_type = other DNA
atcactttctgtcaattgtcttaat

SEQ ID NO: 72 - DNA, 24 bp, synthetic construct
  misc_feature 1..24: note = 4_TGAL2_R
  source 1..24: mol_type = other DNA
gcgataccgatttagctagtattc

SEQ ID NO: 73 - DNA, 48 bp, synthetic construct
  misc_feature 1..48: note = 5_DW_MCH4_F1
  source 1..48: mol_type = other DNA
gaatactagctaaatcggtatcgctgtgtcattgtttgtatggtttag

SEQ ID NO: 74 - DNA, 51 bp, synthetic construct
  misc_feature 1..51: note = 5_DW_MCH4_F2
  source 1..51: mol_type = other DNA
ctatccctttccattatcaactgcttgtcattgtttgtatggtttaggact

SEQ ID NO: 75 - DNA, 25 bp, synthetic construct
  misc_feature 1..25: note = 5_DW_MCH4_R
  source 1..25: mol_type = other DNA
gtcaacaaatctgacatccaatatc

SEQ ID NO: 76 - DNA, 65 bp, synthetic construct
  misc_feature 1..65: note = MCH4_sgRNA-1R
  source 1..65: mol_type = other DNA
aacttgctatttctagctctaaaactggctacttctgcggtaacatgcgcaagcccggaatcgaa

SEQ ID NO: 77 - DNA, 22 bp, synthetic construct
  misc_feature 1..22: note = 1_UP_JEN2-1_F
  source 1..22: mol_type = other DNA
gataggttcaaagccctcgtcg

SEQ ID NO: 78 - DNA, 48 bp, synthetic construct
  misc_feature 1..48: note = 1_UP_JEN2-1_R1
  source 1..48: mol_type = other DNA
gaagtgatgtagatacgccaacaggggttgtgtttcaagcacctgact

SEQ ID NO: 79 - DNA, 23 bp, synthetic construct
  misc_feature 1..23: note = 1_UP_JEN2-1_R2
  source 1..23: mol_type = other DNA
ggttgtgtttcaagcacctgact

SEQ ID NO: 80 - DNA, 57 bp, synthetic construct
  misc_feature 1..57: note = 3_PkPYC1_F
  source 1..57: mol_type = other DNA
caaaacacacaaacaaacacaattacaaaaaatgtcaactgtggaagatcactcctc

SEQ ID NO: 81 - DNA, 50 bp, synthetic construct
  misc_feature 1..50: note = 3_PkPYC1_R
  source 1..50: mol_type = other DNA
attaagacaattgacagaaagtgatttaagctgctggcgcttcatctttg

SEQ ID NO: 82 - DNA, 53 bp, synthetic construct
  misc_feature 1..53: note = 3_AoPYC_F
  source 1..53: mol_type = other DNA
caaaacacacaaacaaacacaattacaaaaaatggctgcaccattcagacaac

SEQ ID NO: 83 - DNA, 50 bp, synthetic construct
  misc_feature 1..50: note = 3_AoPYC_R
  source 1..50: mol_type = other DNA
attaagacaattgacagaaagtgatttaagccttaacaatcttacaaacc

SEQ ID NO: 84 - DNA, 49 bp, synthetic construct
  misc_feature 1..49: note = 5_DW_JEN2-1_F1
  source 1..49: mol_type = other DNA
gaatactagctaaatcggtatcgcccacacccctgtggacctgttctat

SEQ ID NO: 85 - DNA, 48 bp, synthetic construct
  misc_feature 1..48: note = 5_DW_JEN2-1_F2
  source 1..48: mol_type = other DNA
agtcaggtgcttgaaacacaaccccctgtggacctgttctatgtaaac

SEQ ID NO: 86 - DNA, 23 bp, synthetic construct
  misc_feature 1..23: note = 5_DW_JEN2-1_R
  source 1..23: mol_type = other DNA
attcctcccatttctaccccctg

SEQ ID NO: 87 - DNA, 65 bp, synthetic construct
  misc_feature 1..65: note = JEN2-1_sgRNA-1R
  source 1..65: mol_type = other DNA
aacttgctatttctagctctaaaactcaagtgttcattattgtgatgcgcaagcccggaatcgaa

SEQ ID NO: 88 - DNA, 26 bp, synthetic construct
  misc_feature 1..26: note = 1_UP_PPDC1_F
  source 1..26: mol_type = other DNA
gtatcctctatcgtatcgtatcgtag

SEQ ID NO: 89 - DNA, 48 bp, synthetic construct
  misc_feature 1..48: note = 1_UP_PPDC1_R
  source 1..48: mol_type = other DNA
gaagtgatgtagatacgccaacaggccatcgtatcatttgtagcccac

SEQ ID NO: 90 - DNA, 55 bp, synthetic construct
  misc_feature 1..55: note = 3_PkFUM1_F
  source 1..55: mol_type = other DNA
caaaacacacaaacaaacacaattacaaaaaatgttctcaactacctcaattgca

SEQ ID NO: 91 - DNA, 52 bp, synthetic construct
  misc_feature 1..52: note = 3_PkFUM1_R
  source 1..52: mol_type = other DNA
attaagacaattgacagaaagtgatctaatcctttggaccaatcatgttttc

SEQ ID NO: 92 - DNA, 53 bp, synthetic construct
  misc_feature 1..53: note = 5_DW_PPDC1_F
  source 1..53: mol_type = other DNA
gaatactagctaaatcggtatcgctgacatctgaatgtaaaatgaacattaaa

SEQ ID NO: 93 - DNA, 23 bp, synthetic construct
  misc_feature 1..23: note = 5_DW_PPDC1_R
  source 1..23: mol_type = other DNA
gcaaagacgcaatattctctctc

SEQ ID NO: 94 - DNA, 65 bp, synthetic construct
  misc_feature 1..65: note = PPDC1_sgRNA-1R
  source 1..65: mol_type = other DNA
aacttgctatttctagctctaaaactgtcctttttatacgccttctgcgcaagcccggaatcgaa

SEQ ID NO: 95 - protein, 485 aa, Pichia kudriavzevii
MLAARSLKARMSTRAFSTTSIAKRIEKDAFGDIEVPNEKYWGAQTQRSLQNFKIGGKREVMPEPIIKSFGILKKATAKINAESGALDPKLSEAIQQAATEVYEGKLMDHFPLVVFQTGSGTQSNMNANEVISNRAIEILGGELGSKTPVHPNDHVNMSQSSNDTFPTVMHIAAVTEVSSHLLPELTALRDALQKKSDEFKNIIKIGRTHLQDATPLTLGQEFSGYVQQCTNGIKRIEIALEHLRYLAQGGTAVGTGLNTKKGFAEKVANEVTKLTGLQFYTAPNKFEALAAHDAVVEMSGALNTVAVSLFKIAQDIRYLGSGPRCGYGELALPENEPGSSIMPGKVNPTQNEALTMLCTQVFGNHSCITFAGASGQFELNVFKPVMISNLLSSIRLLGDGCNSFRIHCVEGIIANTDKIDKLLHESLMLVTALNPHIGYDKASKIAKNAHKKGLTLKQSALELGYLTEEQFNEWVRPENMIGPKD

SEQ ID NO: 96 - DNA, 546 bp, synthetic construct
  misc_feature 1..546: note = PDC1_sgRNA_1
  source 1..546: mol_type = other DNA
caaggatcttaccgctgttgagatccagttcgatgtaacccactcgtgcacccaactgatcttcagcatcttttactttcaccagcgtttctgggtgagcaaaaacaggaaggcaaaatgccgcaaaaaagggaataagggcgacacggaaatgttgaatactcatactcttcctttttcaatattattgaagcatttatcagggttattgtctcatgagcggatacatatttgaatgtatttagaaaaataaacaaataggggttccgcgcacatttccccgaaaagtgccacctgacgtcccaatgattttaactttctccttgaacttctgtctaaccttctacaatcttcttcaagcttctatttgatttctcaaatcaaagatagaaaaagagtattttgtctaatctctaaaaaatcaatacaagcgcaagtggtttagtggtaaaattcaacgttgccatcgttgagcccctggttcgattccgggcttgcgcaaacgctaacgagttgaatgcgttttagagctagaaatagcaagtt

SEQ ID NO: 97 - DNA, 500 bp, synthetic construct
  misc_feature 1..500: note = sgRNA_2
  source 1..500: mol_type = other DNA
gttttagagctagaaatagcaagttaaaataaggctagtccgttatcaacttgaaaaagtggcaccgagtcggtgctttttttatcggaaagaacatgtgagcaaaaggccggttagacctagttcaaaagccaaagtgcctaattcctctagaaaatgtgtagatttcagattcgaaacccaagtttggcggcccaaaaaaaccattcaatccactcggccacgcaagtttcaaaggtggcaaaaaaaaatgcggtaataacaatcatttattaatcacgtgattgcaagagtgttaaaatgaaatttgaaaaaaaaaaggattgtcttatcttaaccacaaccacatagaggcttgggagattttgtttagcaacaaattttgagaaaaactagtactctaaaagcttcttgtctttgcaaggagagaatttacagcaaatttgtcttaacctcttttgaatttgataacttcttaccagaataatatgcagtttgct

SEQ ID NO: 98 - DNA, 1401 bp, synthetic construct
  misc_feature 1..1401: note = encoding EcSthA
  source 1..1401: mol_type = other DNA
atgccacactcttatgattacgacgctattgttatcggttccggtccaggtggtgaaggtgcagctatgggtttagtcaagcaaggtgctagagttgcagttattgaaagataccaaaacgttggtggtggttgtactcactggggtactattccatccaaggctttgagacatgctgtttccagaatcatcgaatttaaccaaaacccattgtactccgatcactccagattgttaagatcctctttcgctgatattttgaaccatgcagacaacgttattaaccaacaaactagaatgagacaaggtttctacgaaagaaaccactgtgaaattttgcaaggtaacgctagatttgttgacgaacataccttggcattagattgtccagacggttccgttgaaactttaaccgctgaaaagttcgttattgcatgtggttccagaccataccacccaactgatgttgactttacccatccaagaatttacgattctgactccattttgtccatgcaccatgaaccaagacacgttttaatttacggtgctggtgttattggttgtgaatacgcatctattttcagaggtatggatgttaaggttgacttgattaacactagagatagattgttagctttcttggatcaagaaatgtctgactccttatcttaccacttttggaactctggtgttgttatcagacataacgaagaatacgaaaagattgaaggttgtgatgacggtgttattatgcatttgaagtccggtaagaagttaaaggctgactgtttgttatacgcaaacggtagaactggtaacaccgattctttggcattacaaaacattggtttggaaactgactccagaggtcaattaaaggttaactctatgtaccaaaccgctcaaccacacgtttacgcagttggtgatgttattggttacccatccttggcttctgctgcatacgaccaaggtagaattgctgcacaagcattggttaagggtgaagctactgcacatttgatcgaagatattccaactggtatctacaccattccagaaatttcttccgttggtaaaactgaacaacaattgaccgctatgaaggttccatacgaagttggtagagcacaatttaagcacttagctagagcacaaattgttggtatgaacgttggtactttgaagattttattccacagagaaaccaaggaaattttaggtattcattgtttcggtgaaagagctgctgaaatcatccatatcggtcaagctatcatggaacaaaagggtggtggtaacaccattgaatacttcgttaacactacctttaactacccaactatggcagaagcatacagagtcgcagcattgaacggtttgaacagattattttaa

SEQ ID NO: 99 - DNA, 993 bp, synthetic construct
  misc_feature 1..993: note = encoding AoMDH
  source 1..993: mol_type = other DNA
atggttaaggctgcagttttaggtgcttctggtggtattggtcaaccattatccttgttattgaagacctgtccattggttgaagaattagctttgtacgatgttgttaacactccaggtgttgctgcagacttatctcacatttcttccattgcaaagatttccggtttcttgccaaaggatgacggtttaaagcaagctttgaccggtgcaaacattgttgttattccagctggtattccaagaaagcctggtatgactagagatgatttgttcaagattaacgcaggtattgttagagatttggttaagggtattgctgaattctgtccaaaggcattcgttttagttatttctaacccagttaactccaccgttccaattgctgcagaagttttgaaggctgcaggtgttttcgatccaaagagattatttggtgttactaccttggacgttgttagagctgaaactttcacccaagaattttctggtcaaaaggatccatccgcagttcaaattccagttgttggtggtcactctggtgaaaccattgttccattattctccaagactaccccagctattcaaattccagaagaaaagtacgacgcattgattcatagagttcaatttggtggtgacgaagttgttcaagcaaaggacggtgctggttctgcaactttatccatggcttacgcaggttacagattcgctgaatctgttattaaggcatccaagggtcaaaccggtattgttgaaccaacttttgtttacttgccaggtattccaggtggtgacgaaattgttaaggctactggtgttgaattcttttctactttggttaccttgggtactaacggtgctgaaaaggcatccaacgttttagaaggtgttaccgaaaaggaaaagaagttattggaagcatgtactaagggtttgaagggtaacattgaaaagggtattgacttcgttaagaacccaccaccaaagtaa

SEQ ID NO: 100 - DNA, 630 bp, Pichia kudriavzevii
  misc_feature 1..630: note = PkENO1 promoter
  source 1..630: mol_type = other DNA
caacaacacttcgccaaagacaccctttccagggaggatccactcccaacgtctctccataatgtctctgttggcccatgtctctgtcgttgacaccgtaaccacaccaaccaacccgtccattgtactgggatggtcgtccatagacacctctccaacggggaacacctcattcgtaaaccgccaaggttaccgttcctcctgactcgccccgttgttgatgctgcgcacctgtggttgcccaacatggttgtatatcgtgtaaccacaccaacacatgtgcagcacatgtgtttaaaagagtgtcatggaggtggatcatgatggaagtggactttaccacttgggaactgtctccactcccgggaagaaaagacccggcgtatcacgcggttgcctcaatggggcaatttggaaggagaaatatagggaaaatcacgtcgctctcggacggggaagagttccagactatgaggggggggggtggtatataaagacaggagatgtccacccccagagagaggaagaagttggaactttagaagagagagataactttccccagtgtccatcaatacacaaccaaacacaaactctatatttacacatataaccccctccaaccaaaca

SEQ ID NO: 101 - DNA, 501 bp, Pichia kudriavzevii
  misc_feature 1..501: note = PkSED1 terminator
  source 1..501: mol_type = other DNA
gtggattaggttactgctctttcttttggtaatttataatttaaacaagtttatttaatttgaaactcttatttacttagattagattttaaacttacatacttttaataactctgggatatcctatttaatataactaatagctaatttgttctttttcagttgaatcttttggcgattctctctctcccttttctgttctttaacatctttaccgtaaagtattggaataaagtaatgtttgcaattagggaggtccataaaaaaatcgacccgtcgccttttcttttattcttacccatcgcgctgctataattgcaaagttcccctgtgtttgttgtattcgtttgtatttgtagaggtgtactcaatgtcgaaatctccactgtttctgtttttgctctcaaagagaaatcaaacaatgtccttcaacgtgttcaacgacggtagagtgtcccggaaattacatcgcatctctcaactataccaaatccaaccaag

SEQ ID NO: 102 - DNA, 49 bp, synthetic construct
  misc_feature 1..49: note = 3_EcSthA_F
  source 1..49: mol_type = other DNA
actaccacccccaacacaaacacaatgccacactcttatgattacgacg

SEQ ID NO: 103 - DNA, 55 bp, synthetic construct
  misc_feature 1..55: note = 3_EcSthA_R
  source 1..55: mol_type = other DNA
cccttgaacaaacatcttgttgtagttaaaataatctgttcaaaccgttcaatgc

SEQ ID NO: 104 - DNA, 25 bp, synthetic construct
  misc_feature 1..25: note = 1_UP_UGA2_F
  source 1..25: mol_type = other DNA
tgcagtcacacatacacattaagcg

SEQ ID NO: 105 - DNA, 49 bp, synthetic construct
  misc_feature 1..49: note = 1_UP_UGA2_R1
  source 1..49: mol_type = other DNA
ggtgtctttggcgaagtgttgttgggtagctgtgaggaacgattactac

SEQ ID NO: 106 - DNA, 25 bp, synthetic construct
  misc_feature 1..25: note = 1_UP_UGA2_R2
  source 1..25: mol_type = other DNA
ggtagctgtgaggaacgattactac

SEQ ID NO: 107 - DNA, 23 bp, synthetic construct
  misc_feature 1..23: note = 2_PENO1_F
  source 1..23: mol_type = other DNA
caacaacacttcgccaaagacac

SEQ ID NO: 108 - DNA, 24 bp, synthetic construct
  misc_feature 1..24: note = 2_PENO1_R
  source 1..24: mol_type = other DNA
tgtttggttggagggggttatatg

SEQ ID NO: 109 - DNA, 49 bp, synthetic construct
  misc_feature 1..49: note = 3_AoMDH_F
  source 1..49: mol_type = other DNA
catataaccccctccaaccaaacaatggttaaggctgcagttttaggtg

SEQ ID NO: 110 - DNA, 49 bp, synthetic construct
  misc_feature 1..49: note = 3_AoMDH_R
  source 1..49: mol_type = other DNA
caaaagaaagagcagtaacctaatccacttactttggtggtgggttctt

SEQ ID NO: 111 - DNA, 28 bp, synthetic construct
  misc_feature 1..28: note = 4_TSED1_F
  source 1..28: mol_type = other DNA
gtggattaggttactgctctttcttttg

SEQ ID NO: 112 - DNA, 25 bp, synthetic construct
  misc_feature 1..25: note = 4_TSED1_R
  source 1..25: mol_type = other DNA
cttggttggatttggtatagttgag

SEQ ID NO: 113 - DNA, 50 bp, synthetic construct
  misc_feature 1..50: note = 5_DW_UGA2_F1
  source 1..50: mol_type = other DNA
ctctcaactataccaaatccaaccaaggctagaatcttcagatttggcga

SEQ ID NO: 114 - DNA, 48 bp, synthetic construct
  misc_feature 1..48: note = 5_DW_UGA2_F2
  source 1..48: mol_type = other DNA
gtagtaatcgttcctcacagctaccgctagaatcttcagatttggcga

SEQ ID NO: 115 - DNA, 26 bp, synthetic construct
  misc_feature 1..26: note = 5_DW_UGA2_R
  source 1..26: mol_type = other DNA
caagaatatgtgattcatgatggtgg

SEQ ID NO: 116 - DNA, 65 bp, synthetic construct
  misc_feature 1..65: note = UGA2_sgRNA-1R
  source 1..65: mol_type = other DNA
aacttgctatttctagctctaaaacttgactagggcaccggttcttgcgcaagcccggaatcgaa

SEQ ID NO: 117 - DNA, 789 bp, Pichia kudriavzevii
  misc_feature 1..789: note = encoding PkURA3
  source 1..789: mol_type = other DNA
atggcgtcatacaaagaaagatcagaatcacacacttcccctgttgctaggagacttttctccatcatggaggaaaagaagtctaacctttgtgcatcattggatattactgaaactgaaaagcttctctctattttggacactattggtccttacatctgtctagttaaaacacacatcgatattgtttctgattttacgtatgaaggaactgtgttgcctttgaaggagcttgccaagaaacataattttatgatttttgaagatagaaaatttgctgatattggtaacactgttaaaaatcaatataaatctggtgtcttccgtattgccgaatgggctgacatcactaatgcacatggtgtaacgggtgcaggtattgtttctggcttgaaggaggccgcccaagaaacaaccagtgaacctagaggtttgctaatgcttgctgagttatcatcaaagggttctttagcatatggtgaatatacagaaaaaacagtagaaattgctaaatctgataaagagtttgtcattggttttattgcgcaacacgatatgggcggtagagaagaaggttttgactggatcattatgactccaggggttggtttagatgacaaaggtgatgcacttggtcaacaatatagaactgttgatgaagttgtaaagactggaacggatatcataattgttggtagaggtttgtatggtcaaggaagagatcctgtagagcaagctaaaagataccaacaagctggttggaatgcttatttaaacagatttaaatga

SEQ ID NO: 118 - DNA, 632 bp, Pichia kudriavzevii
  misc_feature 1..632: note = PkURA3 promoter
  source 1..632: mol_type = other DNA
ggtatagtccgtcagttatattggaagataataagaaaagaatatcaaaactatttaattagttaattgtataaactgtatgtcattataaacagggaaggttgacattgtctagcggcaatcattgtctcatttggttcattaacttttggttctgttcttggaaacgggtaccaactctctcagagtgcttcaaaaatttttcagcacatttggttagacatgaactttctctgctggttaaggattcagaggtgaagtcttgaacacaatcgttgaaacatctgtccacaagagatgtgtatagcctcatgaaatcagccatttgcttttgttcaacgatcttttgaaattgttgttgttcttggtagttaagttgatccatcttggcttatgttgtgtgtatgttgtagttattcttagtatattcctgtcctgagtttagtgaaacataatatcgccttgaaatgaaaatgctgaaattcgtcgacatacaatttttcaaactttttttttttcttggtgcacggacatgtttttaaaggaagtactctataccagttattcttcacaaatttaattgctggagaatagatcttcaacgctttaataaagtagtttgtttgtcaagg

SEQ ID NO: 119 - DNA, 493 bp, Pichia kudriavzevii
  misc_feature 1..493: note = PkURA3 terminator
  source 1..493: mol_type = other DNA
ttcttacacaaagatttgatacatgtacactagtttaaataagcatgaaaagaattacacaagcaaaaaaaaaattaaatgaggtactttacgttcacctacaaccaaaaaaactagatagagtaaaatcttatgatttagaaaaagttgtttaacaaaggctttagtatgtgaatttttaatgtagcaaagcgataactaataaacataaacaaaagtatggttttctttatcagtcaaatcattatcgattgattgttccgcgtattctaagtgttttatatcattcatagttaacgattgcttttgtttattctgtattctcagcataagatagtaaaggataccggtgaacgccataattgaaaaggaagcttccatggcatgtatccccatcggatactttggtgcttgagaacctttgaaaaaatatggaccgataatgttaccaactgcataccaaactgcaacagaaacatacatgaacgtcttc

SEQ ID NO: 120 - DNA, 26 bp, synthetic construct
  misc_feature 1..26: note = 1_UP_JEN2-2_F
  source 1..26: mol_type = other DNA
ccttggaccaaccaataacctgattc

SEQ ID NO: 121 - DNA, 56 bp, synthetic construct
  misc_feature 1..56: note = 1_UP_JEN2-2_R1
  source 1..56: mol_type = other DNA
cttccaatataactgacggactataccttgctatcttttggtattgtgcataatca

SEQ ID NO: 122 - DNA, 29 bp, synthetic construct
  misc_feature 1..29: note = 1_UP_JEN2-2_R2
  source 1..29: mol_type = other DNA
ttgctatcttttggtattgtgcataatca

SEQ ID NO: 123 - DNA, 28 bp, synthetic construct
  misc_feature 1..28: note = 2_PkURA3_F
  source 1..28: mol_type = other DNA
ggtatagtccgtcagttatattggaaga

SEQ ID NO: 124 - DNA, 26 bp, synthetic construct
  misc_feature 1..26: note = 2_PkURA3_R
  source 1..26: mol_type = other DNA
gaagacgttcatgtatgtttctgttg

SEQ ID NO: 125 - DNA, 49 bp, synthetic construct
  misc_feature 1..49: note = 3_DW_JEN2-2_F1
  source 1..49: mol_type = other DNA
caacagaaacatacatgaacgtcttccagcaatgttaaccccagaagct

SEQ ID NO: 126 - DNA, 48 bp, synthetic construct
  misc_feature 1..48: note = 3_DW_JEN2-2_F2
  source 1..48: mol_type = other DNA
tatgcacaataccaaaagatagcaacagcaatgttaaccccagaagct

SEQ ID NO: 127 - DNA, 25 bp, synthetic construct
  misc_feature 1..25: note = 3_DW_JEN2-2_R
  source 1..25: mol_type = other DNA
gcagtttctgcaagatttcacacag

SEQ ID NO: 128 - DNA, 65 bp, synthetic construct
  misc_feature 1..65: note = JEN2-2_sgRNA-1R
  source 1..65: mol_type = other DNA
aacttgctatttctagctctaaaacggcaatggattcaacaaatgtgcgcaagcccggaatcgaa

SEQ ID NO: 129 - DNA, 804 bp, Saccharomyces cerevisiae
  source 1..804: mol_type = other DNA
atgtcgaaagctacatataaggaacgtgctgctactcatcctagtcctgttgctgccaagctatttaatatcatgcacgaaaagcaaacaaacttgtgtgcttcattggatgttcgtaccaccaaggaattactggagttagttgaagcattaggtcccaaaatttgtttactaaaaacacatgtggatatcttgactgatttttccatggagggcacagttaagccgctaaaggcattatccgccaagtacaattttttactcttcgaagacagaaaatttgctgacattggtaatacagtcaaattgcagtactctgcgggtgtatacagaatagcagaatgggcagacattacgaatgcacacggtgtggtgggcccaggtattgttagcggtttgaagcaggcggcggaagaagtaacaaaggaacctagaggccttttgatgttagcagaattgtcatgcaagggctccctagctactggagaatatactaagggtactgttgacattgcgaagagcgacaaagattttgttatcggctttattgctcaaagagacatgggtggaagagatgaaggttacgattggttgattatgacacccggtgtgggtttagatgacaagggagacgcattgggtcaacagtatagaaccgtggatgatgtggtctctacaggatctgacattattattgttggaagaggactatttgcaaagggaagggatgctaaggtagagggtgaacgttacagaaaagcaggctgggaagcatatttgagaagatgcggccagcaaaactaa

SEQ ID NO: 130 - DNA, 902 bp, Saccharomyces cerevisiae
  source 1..902: mol_type = other DNA
acgtacggtcaagaagacatatttgacctcttaacaggttcagacgcgactgcctcatcagtaagacccgttgaaaagaacttacctgaaaaaaacgaatatatactagcgttgaatgttagcgtcaacaacaagaagtttaatgacgcggaggccaaggcaaaaagattccttgattacgtaagggagttagaatcattttgaataaaaaacacgctttttcagttcgagtttatcattatcaatactgccatttcaaagaatacgtaaataattaatagtagtgattttcctaactttatttagtcaaaaaattagccttttaattctgctgtaacccgtacatgcccaaaatagggggcgggttacacagaatatataacatcgtaggtgtctgggtgaacagtttattcctggcatccactaaatataatggagcccgctttttaagctggcatccagaaaaaaaaagaatcccagcaccaaaatattgttttcttcaccaaccatcagttcataggtccattctcttagcgcaactacagagaacaggggcacaaacaggcaaaaaacgggcacaacctcaatggagtgatgcaacctgcctggagtaaatgatgacacaaggcaattgacccacgcatgtatctatctcattttcttacaccttctattaccttctgctctctctgatttggaaaaagctgaaaaaaaaggttgaaaccagttccctgaaattattcccctacttgactaataagtatataaagacggtaggtattgattgtaattctgtaaatctatttcttaaacttcttaaattctacttttatagttagtcttttttttagttttaaaacaccaagaacttagtttcgaataaacacacataaacaaacaaa

SEQ ID NO: 131 - DNA, 556 bp, Saccharomyces cerevisiae
  source 1..556: mol_type = other DNA
tgcgtttgaagtgagacgctccatcatctctcttaatttttcatgactgacgttttttcttcattttaattatcatagtatttgtttgaaaaaaaaaaaaaaaaatttcccttatcaatgatatccttacgattatataaattccttacctaaacctattatttgtgtacatatatcagagtattattacatatataacctttttctctaaaacaggaaaaaaaaaagaaaacgataacatgctctgccatcctttgttcaccgagcaaaattaaaaacgcaaaatgaattgtccctatgaaattattaaaggaccacatcaccagacttatctctggggggtcctctagaaaataagtcaggtacttgcctggactttcttccagttgaattcctgagctaacatacaattaatggagtgagaatgttcgaacgatccaggagttgcttttttcagtcatttgtttatcagtgtaacaagcatttcctttatttcttttatatcaacctgcaacctattaatattcaattcaacgtctcggagcttttctcgtac

SEQ ID NO: 132 - DNA, 519 bp, Saccharomyces cerevisiae
  source 1..519: mol_type = other DNA
gtattgagaagggcaacggttcatcatctcatggatctgcacatgaacaaacaccagagtcaaacgacgttgaaattgaggctactgcgccaattgatgacaatacagacgatgataacaaaccgaagttatctgatgtagaaaaggattaaagatgctaagagatagtgatgatatttcataaataatgtaattctatatatgttaattaccttttttgcgaggcatatttatggtgaaggataagttttgaccatcaaagaaggttaatgtggctgtggtttcagggtccataaagcttttcaattcatcttttttttttttgttcttttttttgattccggtttctttgaaatttttttgattcggtaatctccgagcagaaggaagaacgaaggaaggagcacagacttagattggtatatatacgcatatgtggtgttgaagaaacatgaaattgcccagtattcttaacccaactgcacagaacaaaaacctgcaggaaacgaagataaatca

SEQ ID NO: 133 - DNA, 541 bp, Saccharomyces cerevisiae
  source 1..541: mol_type = other DNA
acggtggtgtttgacacatccgccttcttaatgctttctttcagtattatgttatttttttgttattcgtttttcacttctaggctttttgacagactagccccgttataccaccatctttgtgggaaagcccctaaattgccctgagcagtatcgtttcatgtctagtctctttaaagatgtttcttacgcgttgcgtgtaaaacatcctctcattcaagacagggttttctaaaagcaataggggtagtttaataattcttatataatcatcatatacactatttttagttcttaattctttaatacaaacttattaatgtgctctccattgatctcttaatcaggaggcgatatataccggaagcggtgtacttttcttcacctcttactcaactatgttgatgtgcaagtttaaccactcgtcgatattatctattgctataacgaaaactttattcgagttcacagtgaaaaacttcagcacatttatggaagatctaagcaaaatggagaacgccagtagatgcgaacaacaaac

SEQ ID NO: 134 - DNA, 25 bp, synthetic construct
  source 1..25: mol_type = other DNA
gtattgagaagggcaacggttcatc

SEQ ID NO: 135 - DNA, 45 bp, synthetic construct
  source 1..45: mol_type = other DNA
gcggatgtgtcaaacaccaccgttagttttgctggccgcatcttc

SEQ ID NO: 136 - DNA, 21 bp, synthetic construct
  source 1..21: mol_type = other DNA
acggtggtgtttgacacatcc

SEQ ID NO: 137 - DNA, 48 bp, synthetic construct
  source 1..48: mol_type = other DNA
caaatatgtcttcttgaccgtacgtgtttgttgttcgcatctactggc

SEQ ID NO: 138 - DNA, 23 bp, synthetic construct
  source 1..23: mol_type = other DNA
gtttgttgttcgcatctactggc

SEQ ID NO: 139 - DNA, 25 bp, synthetic construct
  source 1..25: mol_type = other DNA
acgtacggtcaagaagacatatttg

SEQ ID NO: 140 - DNA, 26 bp, synthetic construct
  source 1..26: mol_type = other DNA
tttgtttgtttatgtgtgtttattcg

SEQ ID NO: 141 - DNA, 51 bp, synthetic construct
  source 1..51: mol_type = other DNA
cgaataaacacacataaacaaacaaaatgggtttgtctaccgcatactctc

SEQ ID NO: 142 - DNA, 49 bp, synthetic construct
  source 1..49: mol_type = other DNA
gatggagcgtctcacttcaaacgcattaaacttcacctggcaacatagt

SEQ ID NO: 143 - DNA, 25 bp, synthetic construct
  source 1..25: mol_type = other DNA
tgcgtttgaagtgagacgctccatc

SEQ ID NO: 144 - DNA, 25 bp, synthetic construct
  source 1..25: mol_type = other DNA
gtacgagaaaagctccgagacgttg

SEQ ID NO: 145 - DNA, 54 bp, synthetic construct
  source 1..54: mol_type = other DNA
caacgtctcggagcttttctcgtacgcatgtatactaaactcacaaattagagc

SEQ ID NO: 146 - DNA, 52 bp, synthetic construct
  source 1..52: mol_type = other DNA
gccagtagatgcgaacaacaaacgcatgtatactaaactcacaaattagagc

SEQ ID NO: 147 - DNA, 23 bp, synthetic construct
  source 1..23: mol_type = other DNA
tacaccttatcggcccaagcctt

SEQ ID NO: 148 - DNA, 1218 bp, Yarrowia lipolytica
  source 1..1218: mol_type = other DNA
atggaacccgaaactaagaagaccaagactgactccaagaagattgttcttctcggcggcgacttctgtggccccgaggtgattgccgaggccgtcaaggtgctcaagtctgttgctgaggcctccggcaccgagtttgtgtttgaggaccgactcattggaggagctgccattgagaaggagggcgagcccatcaccgacgctactctcgacatctgccgaaaggctgactctattatgctcggtgctgtcggaggcgctgccaacaccgtatggaccactcccgacggacgaaccgacgtgcgacccgagcagggtctcctcaagctgcgaaaggacctgaacctgtacgccaacctgcgaccctgccagctgctgtcgcccaagctcgccgatctctcccccatccgaaacgttgagggcaccgacttcatcattgtccgagagctcgtcggaggtatctactttggagagcgaaaggaggatgacggatctggcgtcgcttccgacaccgagacctactccgttcctgaggttgagcgaattgcccgaatggccgccttcctggcccttcagcacaacccccctcttcccgtgtggtctcttgacaaggccaacgtgctggcctcctctcgactttggcgaaagactgtcactcgagtcctcaaggacgaattcccccagctcgagctcaaccaccagctgatcgactcggccgccatgatcctcatcaagcagccctccaagatgaatggtatcatcatcaccaccaacatgtttggcgatatcatctccgacgaggcctccgtcatccccggttctctgggtctgctgccctccgcctctctggcttctctgcccgacaccaacgaggcgttcggtctgtacgagccctgtcacggatctgcccccgatctcggcaagcagaaggtcaaccccattgccaccattctgtctgccgccatgatgctcaagttctctcttaacatgaagcccgccggtgacgctgttgaggctgccgtcaaggagtccgtcgaggctggtatcactaccgccgatatcggaggctcttcctccacctccgaggtcggagacttgttgccaacaaggtcaaggagctgctcaagaaggagtaagtcgtttctacgacgcattgatggaaggagcaaactgacgcgcctgcgggttggtctaccggcagggtccgctagtgtataa

SEQ ID NO: 149 - DNA, 928 bp, Yarrowia lipolytica
  source 1..928: mol_type = other DNA
agtaggatgtcctgcacgggtctttttgtggggtgtggagaaaggggtgcttggagatggaagccggtagaaccgggctgcttggggggatttggggccgctgggctccaaagaggggtaggcatttcgttggggttacgtaattgcggcatttgggtcctgcgcgcatgtcccattggtcagaattagtccggataggagacttatcagccaatcacagcgccggatccacctgtaggttgggttgggtgggagcacccctccacagagtagagtcaaacagcagcagcaacatgatagttgggggtgtgcgtgttaaaggaaaaaaaaagaagcttgggttatattcccgctctatttagaggttgcgggatagacgccgacggagggcaatggcgccatggaaccttgcggatatcgatacgccgcggcggactgcgtccgaaccagctccagcagcgttttttccgggccattgagccgactgcgaccccgccaacgtgtcttggcccacgcactcatgtcatgttggtgttgggaggccactttttaagtagcacaaggcacctagctcgcagcaaggtgtccgaaccaaagaagcggctgcagtggtgcaaacggggcggaaacggcgggaaaaagccacgggggcacgaattgaggcacgccctcgaatttgagacgagtcacggccccattcgcccgcgcaatggctcgccaacgcccggtcttttgcaccacatcaggttaccccaagccaaacctttgtgttaaaaagcttaacatattataccgaacgtaggtttgggcgggcttgctccgtctgtccaaggcaacatttatataagggtctgcatcgccggctcaattgaatcttttttcttcttctcttctctatattcattcttgaattaaacacacatcaaca

SEQ ID NO: 150 - DNA, 563 bp, Yarrowia lipolytica
  source 1..563: mol_type = other DNA
taggtgtacaatagtgaaggaaacagagttaataaatatatacaattagtgtacgtacatctggtagaacaatgtgttggcataattagggacggtatgaactgagtcctgccaacctgatgctaactaatgtgtggttgtaattggactgggtcgattttcgagaaataaaccaataaacgaacacgttgttcctagcccctttaaagagacagtgcaagtactgtacatactgtacttagaagcatactggtatgtactgtatgtactgtacatgcttcatctggctggatcaaagacgatgatcaatacacagggacccaacgggaatagaaatcacataggtgtacaagtattttataataacaagtaaccaaagaagctgtcttagttggtcggttctagtactccagattggtatgtcccctatgtaatacttacgtcgattttaataaagttcatgcacaccaccatctaacatctcagccaagtttactccacaccattatcattacacacgcagcacttctggtatggcatctctagcaacatttcaggtggag

SEQ ID NO: 151 - DNA, 798 bp, Yarrowia lipolytica
  source 1..798: mol_type = other DNA
ttcgacaccatatcatataaaactaacaatgcattgcttattacgaagactacccgttgctatctccacaccgttatctccacggtccaaaggctgctcaatgtgctgcatacgtaacgtggggtgcaaccttgagcacatagtacttttccgaaaaccggcgataattaagtgtgcactccaacttttcacactgagcgtaaaatgtggagaagaaatcggcactaaaaagtcaggtagactggaaaatgcgccatgaaatgaatatctcttgctacagtaatgcccagcatcgaggggtattgtgtcaccaacactatagtggcagctgaagcgctcgtgattgtagtatgagtctttattggtgatgggaagagttcactcaatattctcgttactgccaaaacaccacggtaatcggccagacaccatggatgtagatcaccaagcctgtgaatgttattcgagctaaaatgcacatggttggtgaaaggagtagttgctgtcgaattccgtcgtcgcctgagtcatcatttatttaccagttggccacaaacccttgacgatctcgtatgtcccctccgacatactcccggccggctggggtacgttcgatagcgctatcggcatcgacaaggtttgggtccctagccgataccgcactacctgagtcacaatcttcggaggtttagtcttccacatagcacgggcaaaagtgcgtatatatacaagagcgtttgccagccacagattttcactccacacaccacatcacacatacaaccacacacatccaca

SEQ ID NO: 152 - DNA, 192 bp, Saccharomyces cerevisiae
  source 1..192: mol_type = other DNA
atctcttctcgagtcatgtaattagttatgtcacgcttacattcacgccctccccccacatccgctctaaccgaaaaggaaggagttagacaacctgaagtctaggtccctatttatttttttatagttatgttagtattaagaacgttatttatatttcaaatttttcttttttttctgtacagacgcgtc

SEQ ID NO: 153 - DNA, 28 bp, synthetic construct
  source 1..28: mol_type = other DNA
agtaggatgtcctgcacgggtctttttg

SEQ ID NO: 154 - DNA, 27 bp, synthetic construct
  source 1..27: mol_type = other DNA
tgttgatgtgtgtttaattcaagaatg

SEQ ID NO: 155 - DNA, 49 bp, synthetic construct
  source 1..49: mol_type = other DNA
tcttgaattaaacacacatcaacaatgggtttgtctaccgcatactctc

SEQ ID NO: 156 - DNA, 50 bp, synthetic construct
  source 1..50: mol_type = other DNA
ctgtttccttcactattgtacacctattaaacttcacctggcaacatagt

SEQ ID NO: 157 - DNA, 26 bp, synthetic construct
  source 1..26: mol_type = other DNA
taggtgtacaatagtgaaggaaacag

SEQ ID NO: 158 - DNA, 26 bp, synthetic construct
  source 1..26: mol_type = other DNA
ctccacctgaaatgttgctagagatg

SEQ ID NO: 159 - DNA, 52 bp, synthetic construct
  source 1..52: mol_type = other DNA
tctctagcaacatttcaggtggagttcgacaccatatcatataaaactaaca

SEQ ID NO: 160 - DNA, 47 bp, synthetic construct
  source 1..47: mol_type = other DNA
ctaattacatgactcgagaagagatttatacactagcggaccctgcc

SEQ ID NO: 161 - DNA, 30 bp, synthetic construct
  source 1..30: mol_type = other DNA
atctcttctcgagtcatgtaattagttatg

SEQ ID NO: 162 - DNA, 24 bp, synthetic construct
  source 1..24: mol_type = other DNA
gacgcgtctgtacagaaaaaaaag